European Patent Specification EP 4 493 226 B1, published September 2, 2026. Title: Modified Muscle-Specific Promoters. Applicant: REGENEXBIO, Inc. Application WO. The sequence listing filed with the application follows.

SEQUENCE LISTING (72 sequences)

SEQ ID NO: 1 - DNA, 328 bp, synthetic construct
  source 1..328: mol_type = other DNA
ggccgtccgccctcggcaccatcctcacgacacccaaatatggcgacgggtgaggaatggtggggagttatttttagagcggtgaggaaggtgggcaggcagcaggtgttggcgctccatatttggcgggagttatttttagagcggaggaatggtggacacccaaatatggcgacggttcctcacccgtcgctaaaaataactccgtgtccgccctcggccggggccgcattcctgggggccgggcggtgctcccgcccgcctcgataaaaggctccggggccggcggcggcccacgagctacccggaggagcgggaggcgccaagc

SEQ ID NO: 2 - DNA, 328 bp, synthetic construct
  source 1..328: mol_type = other DNA
ggccgtccgccctcggcaccatcctcacgacacccaaatatggcgacgggtgaggaatggtggggagttatttttagagcggtgaggaaggtgggcaggcagcaggtgttgggggagttatttttagagcggggagttatttttagagcggaggaatggtggacacccaaatatggcgacggttcctcacggacacccaaatatggcgacgggccctcggccggggccgcattcctgggggccgggcggtgctcccgcccgcctcgataaaaggctccggggccggcggcggcccacgagctacccggaggagcgggaggcgccaagc

SEQ ID NO: 3 - DNA, 328 bp, synthetic construct
  source 1..328: mol_type = other DNA
ggccgtccgccctcggcaccatcctcacgacacccaaatatggcgacgggtgaggaatggtggggagttatttttagagcggtgaggaaggtgggcaggcagcaggtgttggcgctctaaaaataactcccgggagttatttttagagcggaggaatggtggacacccaaatatggcgacggttcctcacccgtcgccatatttgggtgtccgccctcggccggggccgcattcctgggggccgggcggtgctcccgcccgcctcgataaaaggctccggggccggcggcggcccacgagctacccggaggagcgggaggcgccaagc

SEQ ID NO: 4 - DNA, 39 bp, synthetic construct
  source 1..39: mol_type = other DNA
cgctctaaaaaataactcccgggagttatttttagagcg

SEQ ID NO: 5 - DNA, 52 bp, synthetic construct
  source 1..52: mol_type = other DNA
ggacacccaaatatggcgacggttcctcacccgtcgccatatttgggtgtcc

SEQ ID NO: 6 - DNA, 144 bp, synthetic construct
  source 1..144: mol_type = other DNA
ccactacgggtttaggctgcccatgtaaggaggcaaggcctggggacacccgagatgcctggttataattaacccagacatgtggctgccccccccccccccaacacctgctgcctctaaaaataaccctgtccctggtggatc

SEQ ID NO: 7 - DNA, 288 bp, synthetic construct
  source 1..288: mol_type = other DNA
ccactacgggtttaggctgcccatgtaaggaggcaaggcctggggacacccgagatgcctggttataattaacccagacatgtggctgccccccccccccccaacacctgctgcctctaaaaataaccctgtccctggtggatcccactacgggtttaggctgcccatgtaaggaggcaaggcctggggacacccgagatgcctggttataattaacccagacatgtggctgccccccccccccccaacacctgctgcctctaaaaataaccctgtccctggtggatc

SEQ ID NO: 8 - DNA, 432 bp, synthetic construct
  source 1..432: mol_type = other DNA
ccactacgggtttaggctgcccatgtaaggaggcaaggcctggggacacccgagatgcctggttataattaacccagacatgtggctgccccccccccccccaacacctgctgcctctaaaaataaccctgtccctggtggatcccactacgggtttaggctgcccatgtaaggaggcaaggcctggggacacccgagatgcctggttataattaacccagacatgtggctgccccccccccccccaacacctgctgcctctaaaaataaccctgtccctggtggatcccactacgggtttaggctgcccatgtaaggaggcaaggcctggggacacccgagatgcctggttataattaacccagacatgtggctgccccccccccccccaacacctgctgcctctaaaaataaccctgtccctggtggatc

SEQ ID NO: 9 - DNA, 199 bp, synthetic construct
  source 1..199: mol_type = other DNA
cccttcagattaaaaataactgaggtaagggcctgggtaggggaggtggtgtgagacgctcctgtctctcctctatctgcccatcggccctttggggaggaggaatgtgcccaaggactaaaaaaaggccatggagccagaggggcgagggcaacagacctttcatgggcaaaccttggggccctgctgaagctttggc

SEQ ID NO: 10 - DNA, 133 bp, synthetic construct
  source 1..133: mol_type = other DNA
gtaagtatcaaggttacaagacaggtttaaggagaccaatagaaactgggcttgtcgagacagagaagactcttgcgtttctgataggcacctattggtcttactgacatccactttgcctttctctccacag

SEQ ID NO: 11 - DNA, 82 bp, synthetic construct
  source 1..82: mol_type = other DNA
gtgagtatctcagggatccagacatggggatatgggaggtgcctctgatcccagggctcactgtgggtctctctgttcacag

SEQ ID NO: 12 - DNA, 97 bp, synthetic construct
  source 1..97: mol_type = other DNA
gtaagtttagtctttttgtcttttatttcaggtcccggatccggtggtggtgcaaatcaaagaactgctcctcagtggatgttgcctttacttctag

SEQ ID NO: 13 - DNA, 55 bp, synthetic construct
  source 1..55: mol_type = other DNA
ataaaggaaatttattttcattgcaatagtgtgttggaattttttgtgtctctca

SEQ ID NO: 14 - DNA, 127 bp, synthetic construct
  source 1..127: mol_type = other DNA
gatctttttccctctgccaaaaattatggggacatcatgaagccccttgagcatctgacttctggctaataaaggaaatttattttcattgcaatagtgtgttggaattttttgtgtctctcactcg

SEQ ID NO: 15 - protein, 240 aa, synthetic construct
MLWWEEVEDCYEREDVQKKTFTKWVNAQFSKFGKQHIENLFSDLQDGRRLLDLLEGLTGQKLPKEKGSTRVHALNNVNKALRVLQNNNVDLVNIGSTDIVDGNHKLTLGLIWNIILHWQVKNVMKNIMAGLQQTNSEKILLSWVRQSTRNYPQVNVINFTTSWSDGLALNALIHSHRPDLFDWNSVVCQQSATQRLEHAFNIARYQLGIEKLLDPEDVDTTYPDKKSILMYITSLFQVLP

SEQ ID NO: 16 - protein, 12 aa, synthetic construct
QQVSIEAIQEVE

SEQ ID NO: 17 - protein, 75 aa, synthetic construct
MLPRPPKVTKEEHFQLHHQMHYSQQITVSLAQGYERTSSPKPRFKSYAYTQAAYVTTSDPTRSPFPSQHLEAPED

SEQ ID NO: 18 - protein, 9 aa, synthetic construct
KSFGSSLME

SEQ ID NO: 19 - protein, 111 aa, synthetic construct
SEVNLDRYQTALEEVLSWLLSAEDTLQAQGEISNDVEVVKDQFHTHEGYMMDLTAHQGRVGNILQLGSKLIGTGKLSEDEETEVQEQMNLLNSRWECLRVASMEKQSNLHR

SEQ ID NO: 20 - protein, 109 aa, synthetic construct
VLMDLQNQKLKELNDWLTKTEERTRKMEEEPLGPDLEDLKRQVQQHKVLQEDLEQEQVRVNSLTHMVVVVDESSGDHATAALEEQLKVLGDRWANICRWTEDRWVLLQD

SEQ ID NO: 21 - skipped

SEQ ID NO: 22 - protein, 109 aa, synthetic construct
LKWQRLTEEQCLFSAWLSEKEDAVNKIHTTGFKDQNEMLSSLQKLAVLKADLEKKKQSMGKLYSLKQDLLSTLKNKSVTQKTEAWLDNFARCWDNLVQKLEKSTAQISQ

SEQ ID NO: 23 - protein, 47 aa, synthetic construct
QPDLAPGLTTIGASPTQTVTLVTQPVVTKETAISKLEMPSSLMLEVP

SEQ ID NO: 24 - skipped

SEQ ID NO: 25 - protein, 106 aa, synthetic construct
RLQELQEATDELDLKLRQAEVIKGSWQPVGDLLIDSLQDHLEKVKALRGEIAPLKENVSHVNDLARQLTTLGIQLSPYNLSTLEDLNTRWKLLQVAVEDRVRQLHE

SEQ ID NO: 26 - protein, 72 aa, synthetic construct
AHRDFGPASQHFLSTSVQGPWERAISPNKVPYYINHETQTTCWDHPKMTELYQSLADLNNVRFSAYRTAMKL

SEQ ID NO: 27 - protein, 248 aa, synthetic construct
RRLQKALCLDLLSLSAACDALDQHNLKQNDQPMDILQIINCLTTIYDRLEQEHNNLVNVPLCVDMCLNWLLNVYDTGRTGRIRVLSFKTGIISLCKAHLEDKYRYLFKQVASSTGFCDQRRLGLLLHDSIQIPRQLGEVASFGGSNIEPSVRSCFQFANNKPEIEAALFLDWMRLEPQSMVWLPVLHRVAAAETAKHQAKCNICKECPIIGFRYRSLKHFNYDICQSCFFSGRVAKGHKMHYPMVEYC

SEQ ID NO: 28 - protein, 54 aa, synthetic construct
AKHQAKCNICKECPIIGFRYRSLKHFNYDICQSCFFSGRVAKGHKMHYPMVEYC

SEQ ID NO: 29 - protein, 194 aa, synthetic construct
TPTTSGEDVRDFAKVLKNKFRTKRYFAKHPRMGYLPVQTVLEGDNMETPVTLINFWPVDSAPASSPQLSHDDTHSRIEHYASRLAEMENSNGSYLNDSISPNESIDDEHLLIQHYCQSLNQDSPLSQPRSPAQILISLESEERGELERILADLEEENRNLQAEYDRLKQQHEHKGLSPLPSPPEMMPTSPQSPR

SEQ ID NO: 30 - protein, 140 aa, synthetic construct
TPTTSGEDVRDFAKVLKNKFRTKRYFAKHPRMGYLPVQTVLEGDNMETPVTLINFWPVDSAPASSPQLSHDDTHSRIEHYASRLAEMENSNGSYLNDSISPNESIDDEHLLIQHYCQSLNQDSPLSQPRSPAQILISLES

SEQ ID NO: 31 - protein, 4 aa, synthetic construct
ETLE

SEQ ID NO: 32 - skipped

SEQ ID NO: 33 - protein, 35 aa, synthetic construct
MENSNGSYLNDSISPNESIDDEHLLIQHYCQSLNQ

SEQ ID NO: 34 - protein, 3685 aa, Homo sapiens
MLWWEEVEDCYEREDVQKKTFTKWVNAQFSKFGKQHIENLFSDLQDGRRLLDLLEGLTGQKLPKEKGSTRVHALNNVNKALRVLQNNNVDLVNIGSTDIVDGNHKLTLGLIWNIILHWQVKNVMKNIMAGLQQTNSEKILLSWVRQSTRNYPQVNVINFTTSWSDGLALNALIHSHRPDLFDWNSVVCQQSATQRLEHAFNIARYQLGIEKLLDPEDVDTTYPDKKSILMYITSLFQVLPQQVSIEAIQEVEMLPRPPKVTKEEHFQLHHQMHYSQQITVSLAQGYERTSSPKPRFKSYAYTQAAYVTTSDPTRSPFPSQHLEAPEDKSFGSSLMESEVNLDRYQTALEEVLSWLLSAEDTLQAQGEISNDVEVVKDQFHTHEGYMMDLTAHQGRVGNILQLGSKLIGTGKLSEDEETEVQEQMNLLNSRWECLRVASMEKQSNLHRVLMDLQNQKLKELNDWLTKTEERTRKMEEEPLGPDLEDLKRQVQQHKVLQEDLEQEQVRVNSLTHMVVVVDESSGDHATAALEEQLKVLGDRWANICRWTEDRWVLLQDILLKWQRLTEEQCLFSAWLSEKEDAVNKIHTTGFKDQNEMLSSLQKLAVLKADLEKKKQSMGKLYSLKQDLLSTLKNKSVTQKTEAWLDNFARCWDNLVQKLEKSTAQISQAVTTTQPSLTQTTVMETVTTVTTREQILVKHAQEELPPPPPQKKRQITVDSEIRKRLDVDITELHSWITRSEAVLQSPEFAIFRKEGNFSDLKEKVNAIEREKAEKFRKLQDASRSAQALVEQMVNEGVNADSIKQASEQLNSRWIEFCQLLSERLNWLEYQNNIIAFYNQLQQLEQMTTTAENWLKIQPTTPSEPTAIKSQLKICKDEVNRLSDLQPQIERLKIQSIALKEKGQGPMFLDADFVAFTNHFKQVFSDVQAREKELQTIFDTLPPMRYQETMSAIRTWVQQSETKLSIPQLSVTDYEIMEQRLGELQALQSSLQEQQSGLYYLSTTVKEMSKKAPSEISRKYQSEFEEIEGRWKKLSSQLVEHCQKLEEQMNKLRKIQNHIQTLKKWMAEVDVFLKEEWPALGDSEILKKQLKQCRLLVSDIQTIQPSLNSVNEGGQKIKNEAEPEFASRLETELKELNTQWDHMCQQVYARKEALKGGLEKTVSLQKDLSEMHEWMTQAEEEYLERDFEYKTPDELQKAVEEMKRAKEEAQQKEAKVKLLTESVNSVIAQAPPVAQEALKKELETLTTNYQWLCTRLNGKCKTLEEVWACWHELLSYLEKANKWLNEVEFKLKTTENIPGGAEEISEVLDSLENLMRHSEDNPNQIRILAQTLTDGGVMDELINEELETFNSRWRELHEEAVRRQKLLEQSIQSAQETEKSLHLIQESLTFIDKQLAAYIADKVDAAQMPQEAQKIQSDLTSHEISLEEMKKHNQGKEAAQRVLSQIDVAQKKLQDVSMKFRLFQKPANFEQRLQESKMILDEVKMHLPALETKSVEQEVVQSQLNHCVNLYKSLSEVKSEVEMVIKTGRQIVQKKQTENPKELDERVTALKLHYNELGAKVTERKQQLEKCLKLSRKMRKEMNVLTEWLAATDMELTKRSAVEGMPSNLDSEVAWGKATQKEIEKQKVHLKSITEVGEALKTVLGKKETLVEDKLSLLNSNWIAVTSRAEEWLNLLLEYQKHMETFDQNVDHITKWIIQADTLLDESEKKKPQQKEDVLKRLKAELNDIRPKVDSTRDQAANLMANRGDHCRKLVEPQISELNHRFAAISHRIKTGKASIPLKELEQFNSDIQKLLEPLEAEIQQGVNLKEEDFNKDMNEDNEGTVKELLQRGDNLQQRITDERKREEIKIKQQLLQTKHNALKDLRSQRRKKALEISHQWYQYKRQADDLLKCLDDIEKKLASLPEPRDERKIKEIDRELQKKKEELNAVRRQAEGLSEDGAAMAVEPTQIQLSKRWREIESKFAQFRRLNFAQIHTVREETMMVMTEDMPLEISYVPSTYLTEITHVSQALLEVEQLLNAPDLCAKDFEDLFKQEESLKNIKDSLQQSSGRIDIIHSKKTAALQSATPVERVKLQEALSQLDFQWEKVNKMYKDRQGRFDRSVEKWRRFHYDIKIFNQWLTEAEQFLRKTQIPENWEHAKYKWYLKELQDGIGQRQTVVRTLNATGEEIIQQSSKTDASILQEKLGSLNLRWQEVCKQLSDRKKRLEEQKNILSEFQRDLNEFVLWLEEADNIASIPLEPGKEQQLKEKLEQVKLLVEELPLRQGILKQLNETGGPVLVSAPISPEEQDKLENKLKQTNLQWIKVSRALPEKQGEIEAQIKDLGQLEKKLEDLEEQLNHLLLWLSPIRNQLEIYNQPNQEGPFDVKETEIAVQAKQPDVEEILSKGQHLYKEKPATQPVKRKLEDLSSEWKAVNRLLQELRAKQPDLAPGLTTIGASPTQTVTLVTQPVVTKETAISKLEMPSSLMLEVPALADFNRAWTELTDWLSLLDQVIKSQRVMVGDLEDINEMIIKQKATMQDLEQRRPQLEELITAAQNLKNKTSNQEARTIITDRIERIQNQWDEVQEHLQNRRQQLNEMLKDSTQWLEAKEEAEQVLGQARAKLESWKEGPYTVDAIQKKITETKQLAKDLRQWQTNVDVANDLALKLLRDYSADDTRKVHMITENINASWRSIHKRVSEREAALEETHRLLQQFPLDLEKFLAWLTEAETTANVLQDATRKERLLEDSKGVKELMKQWQDLQGEIEAHTDVYHNLDENSQKILRSLEGSDDAVLLQRRLDNMNFKWSELRKKSLNIRSHLEASSDQWKRLHLSLQELLVWLQLKDDELSRQAPIGGDFPAVQKQNDVHRAFKRELKTKEPVIMSTLETVRIFLTEQPLEGLEKLYQEPRELPPEERAQNVTRLLRKQAEEVNTEWEKLNLHSADWQRKIDETLERLQELQEATDELDLKLRQAEVIKGSWQPVGDLLIDSLQDHLEKVKALRGEIAPLKENVSHVNDLARQLTTLGIQLSPYNLSTLEDLNTRWKLLQVAVEDRVRQLHEAHRDFGPASQHFLSTSVQGPWERAISPNKVPYYINHETQTTCWDHPKMTELYQSLADLNNVRFSAYRTAMKLRRLQKALCLDLLSLSAACDALDQHNLKQNDQPMDILQIINCLTTIYDRLEQEHNNLVNVPLCVDMCLNWLLNVYDTGRTGRIRVLSFKTGIISLCKAHLEDKYRYLFKQVASSTGFCDQRRLGLLLHDSIQIPRQLGEVASFGGSNIEPSVRSCFQFANNKPEIEAALFLDWMRLEPQSMVWLPVLHRVAAAETAKHQAKCNICKECPIIGFRYRSLKHFNYDICQSCFFSGRVAKGHKMHYPMVEYCTPTTSGEDVRDFAKVLKNKFRTKRYFAKHPRMGYLPVQTVLEGDNMETPVTLINFWPVDSAPASSPQLSHDDTHSRIEHYASRLAEMENSNGSYLNDSISPNESIDDEHLLIQHYCQSLNQDSPLSQPRSPAQILISLESEERGELERILADLEEENRNLQAEYDRLKQQHEHKGLSPLPSPPEMMPTSPQSPRDAELIAEAKLLRQHKGRLEARMQILEDHNKQLESQLHRLRQLLEQPQAEAKVNGTTVSSPSTSLQRSDSSQPMLLRVVGSQTSDSMGEEDLLSPPQDTSTGLEEVMEQLNNSFPSSRGRNTPGKPMREDTM

SEQ ID NO: 35 - protein, 1337 aa, synthetic construct
MLWWEEVEDCYEREDVQKKTFTKWVNAQFSKFGKQHIENLFSDLQDGRRLLDLLEGLTGQKLPKEKGSTRVHALNNVNKALRVLQNNNVDLVNIGSTDIVDGNHKLTLGLIWNIILHWQVKNVMKNIMAGLQQTNSEKILLSWVRQSTRNYPQVNVINFTTSWSDGLALNALIHSHRPDLFDWNSVVCQQSATQRLEHAFNIARYQLGIEKLLDPEDVDTTYPDKKSILMYITSLFQVLPQQVSIEAIQEVEMLPRPPKVTKEEHFQLHHQMHYSQQITVSLAQGYERTSSPKPRFKSYAYTQAAYVTTSDPTRSPFPSQHLEAPEDKSFGSSLMESEVNLDRYQTALEEVLSWLLSAEDTLQAQGEISNDVEVVKDQFHTHEGYMMDLTAHQGRVGNILQLGSKLIGTGKLSEDEETEVQEQMNLLNSRWECLRVASMEKQSNLHRVLMDLQNQKLKELNDWLTKTEERTRKMEEEPLGPDLEDLKRQVQQHKVLQEDLEQEQVRVNSLTHMVVVVDESSGDHATAALEEQLKVLGDRWANICRWTEDRWVLLQDILLKWQRLTEEQCLFSAWLSEKEDAVNKIHTTGFKDQNEMLSSLQKLAVLKADLEKKKQSMGKLYSLKQDLLSTLKNKSVTQKTEAWLDNFARCWDNLVQKLEKSTAQISQQPDLAPGLTTIGASPTQTVTLVTQPVVTKETAISKLEMPSSLMLEVPTLERLQELQEATDELDLKLRQAEVIKGSWQPVGDLLIDSLQDHLEKVKALRGEIAPLKENVSHVNDLARQLTTLGIQLSPYNLSTLEDLNTRWKLLQVAVEDRVRQLHEAHRDFGPASQHFLSTSVQGPWERAISPNKVPYYINHETQTTCWDHPKMTELYQSLADLNNVRFSAYRTAMKLRRLQKALCLDLLSLSAACDALDQHNLKQNDQPMDILQIINCLTTIYDRLEQEHNNLVNVPLCVDMCLNWLLNVYDTGRTGRIRVLSFKTGIISLCKAHLEDKYRYLFKQVASSTGFCDQRRLGLLLHDSIQIPRQLGEVASFGGSNIEPSVRSCFQFANNKPEIEAALFLDWMRLEPQSMVWLPVLHRVAAAETAKHQAKCNICKECPIIGFRYRSLKHFNYDICQSCFFSGRVAKGHKMHYPMVEYCTPTTSGEDVRDFAKVLKNKFRTKRYFAKHPRMGYLPVQTVLEGDNMETPVTLINFWPVDSAPASSPQLSHDDTHSRIEHYASRLAEMENSNGSYLNDSISPNESIDDEHLLIQHYCQSLNQDSPLSQPRSPAQILISLESEERGELERILADLEEENRNLQAEYDRLKQQHEHKGLSPLPSPPEMMPTSPQSPR

SEQ ID NO: 36 - protein, 1191 aa, synthetic construct
MLWWEEVEDCYEREDVQKKTFTKWVNAQFSKFGKQHIENLFSDLQDGRRLLDLLEGLTGQKLPKEKGSTRVHALNNVNKALRVLQNNNVDLVNIGSTDIVDGNHKLTLGLIWNIILHWQVKNVMKNIMAGLQQTNSEKILLSWVRQSTRNYPQVNVINFTTSWSDGLALNALIHSHRPDLFDWNSVVCQQSATQRLEHAFNIARYQLGIEKLLDPEDVDTTYPDKKSILMYITSLFQVLPQQVSIEAIQEVEMLPRPPKVTKEEHFQLHHQMHYSQQITVSLAQGYERTSSPKPRFKSYAYTQAAYVTTSDPTRSPFPSQHLEAPEDKSFGSSLMESEVNLDRYQTALEEVLSWLLSAEDTLQAQGEISNDVEVVKDQFHTHEGYMMDLTAHQGRVGNILQLGSKLIGTGKLSEDEETEVQEQMNLLNSRWECLRVASMEKQSNLHRVLMDLQNQKLKELNDWLTKTEERTRKMEEEPLGPDLEDLKRQVQQHKVLQEDLEQEQVRVNSLTHMVVVVDESSGDHATAALEEQLKVLGDRWANICRWTEDRWVLLQDILLKWQRLTEEQCLFSAWLSEKEDAVNKIHTTGFKDQNEMLSSLQKLAVLKADLEKKKQSMGKLYSLKQDLLSTLKNKSVTQKTEAWLDNFARCWDNLVQKLEKSTAQISQQPDLAPGLTTIGASPTQTVTLVTQPVVTKETAISKLEMPSSLMLEVPTLERLQELQEATDELDLKLRQAEVIKGSWQPVGDLLIDSLQDHLEKVKALRGEIAPLKENVSHVNDLARQLTTLGIQLSPYNLSTLEDLNTRWKLLQVAVEDRVRQLHEAHRDFGPASQHFLSTSVQGPWERAISPNKVPYYINHETQTTCWDHPKMTELYQSLADLNNVRFSAYRTAMKLRRLQKALCLDLLSLSAACDALDQHNLKQNDQPMDILQIINCLTTIYDRLEQEHNNLVNVPLCVDMCLNWLLNVYDTGRTGRIRVLSFKTGIISLCKAHLEDKYRYLFKQVASSTGFCDQRRLGLLLHDSIQIPRQLGEVASFGGSNIEPSVRSCFQFANNKPEIEAALFLDWMRLEPQSMVWLPVLHRVAAAETAKHQAKCNICKECPIIGFRYRSLKHFNYDICQSCFFSGRVAKGHKMHYPMVEYCTPTTSGEDVRDFAKVLKNKFRTKRYFAKHPRMGYLPVQTVLEGDNMET

SEQ ID NO: 37 - protein, 1283 aa, synthetic construct
MLWWEEVEDCYEREDVQKKTFTKWVNAQFSKFGKQHIENLFSDLQDGRRLLDLLEGLTGQKLPKEKGSTRVHALNNVNKALRVLQNNNVDLVNIGSTDIVDGNHKLTLGLIWNIILHWQVKNVMKNIMAGLQQTNSEKILLSWVRQSTRNYPQVNVINFTTSWSDGLALNALIHSHRPDLFDWNSVVCQQSATQRLEHAFNIARYQLGIEKLLDPEDVDTTYPDKKSILMYITSLFQVLPQQVSIEAIQEVEMLPRPPKVTKEEHFQLHHQMHYSQQITVSLAQGYERTSSPKPRFKSYAYTQAAYVTTSDPTRSPFPSQHLEAPEDKSFGSSLMESEVNLDRYQTALEEVLSWLLSAEDTLQAQGEISNDVEVVKDQFHTHEGYMMDLTAHQGRVGNILQLGSKLIGTGKLSEDEETEVQEQMNLLNSRWECLRVASMEKQSNLHRVLMDLQNQKLKELNDWLTKTEERTRKMEEEPLGPDLEDLKRQVQQHKVLQEDLEQEQVRVNSLTHMVVVVDESSGDHATAALEEQLKVLGDRWANICRWTEDRWVLLQDILLKWQRLTEEQCLFSAWLSEKEDAVNKIHTTGFKDQNEMLSSLQKLAVLKADLEKKKQSMGKLYSLKQDLLSTLKNKSVTQKTEAWLDNFARCWDNLVQKLEKSTAQISQQPDLAPGLTTIGASPTQTVTLVTQPVVTKETAISKLEMPSSLMLEVPTLERLQELQEATDELDLKLRQAEVIKGSWQPVGDLLIDSLQDHLEKVKALRGEIAPLKENVSHVNDLARQLTTLGIQLSPYNLSTLEDLNTRWKLLQVAVEDRVRQLHEAHRDFGPASQHFLSTSVQGPWERAISPNKVPYYINHETQTTCWDHPKMTELYQSLADLNNVRFSAYRTAMKLRRLQKALCLDLLSLSAACDALDQHNLKQNDQPMDILQIINCLTTIYDRLEQEHNNLVNVPLCVDMCLNWLLNVYDTGRTGRIRVLSFKTGIISLCKAHLEDKYRYLFKQVASSTGFCDQRRLGLLLHDSIQIPRQLGEVASFGGSNIEPSVRSCFQFANNKPEIEAALFLDWMRLEPQSMVWLPVLHRVAAAETAKHQAKCNICKECPIIGFRYRSLKHFNYDICQSCFFSGRVAKGHKMHYPMVEYCTPTTSGEDVRDFAKVLKNKFRTKRYFAKHPRMGYLPVQTVLEGDNMETPVTLINFWPVDSAPASSPQLSHDDTHSRIEHYASRLAEMENSNGSYLNDSISPNESIDDEHLLIQHYCQSLNQDSPLSQPRSPAQILISLES

SEQ ID NO: 38 - DNA, 4361 bp, synthetic construct
  source 1..4361: mol_type = other DNA
agaggccgtccgccctcggcaccatcctcacgacacccaaatatggcgacgggtgaggaatggtggggagttatttttagagcggtgaggaaggtgggcaggcagcaggtgttggcgctccatatttggcgggagttatttttagagcggaggaatggtggacacccaaatatggcgacggttcctcacccgtcgctaaaaataactccgtgtccgccctcggccggggccgcattcctgggggccgggcggtgctcccgcccgcctcgataaaaggctccggggccggcggcggcccacgagctacccggaggagcgggaggcgccaagcggaattcgccaccatgctttggtgggaagaggtggaagattgctatgagagggaagatgtgcagaagaaaaccttcaccaaatgggtcaatgcccagttcagcaagtttggcaagcagcacattgagaacctgttcagtgacctgcaggatggcagaaggctgctggatctgctggaaggcctgacaggccagaagctgcctaaagagaagggcagcacaagagtgcatgccctgaacaatgtgaacaaggccctgagagtgctgcagaacaacaatgtggacctggtcaatattggcagcacagacattgtggatggcaaccacaagctgaccctgggcctgatctggaacatcatcctgcactggcaagtgaagaatgtgatgaagaacatcatggctggcctgcagcagaccaactctgagaagatcctgctgagctgggtcagacagagcaccagaaactaccctcaagtgaatgtgatcaacttcaccacctcttggagtgatggactggccctgaatgccctgatccacagccacagacctgacctgtttgactggaactctgttgtgtgccagcagtctgccacacagagactggaacatgccttcaacattgccagataccagctgggaattgagaaactgctggaccctgaggatgtggacaccacctatcctgacaagaaatccatcctcatgtacatcaccagcctgttccaggtgctgccccagcaagtgtccattgaggccattcaagaggttgagatgctgcccagacctcctaaagtgaccaaagaggaacacttccagctgcaccaccagatgcactactctcagcagatcacagtgtctctggcccagggatatgagagaacaagcagccccaagcctaggttcaagagctatgcctacacacaggctgcctatgtgaccacatctgaccccacaagaagcccatttccaagccagcatctggaagcccctgaggacaagagctttggcagcagcctgatggaatctgaagtgaacctggatagataccagacagccctggaagaagtgctgtcctggctgctgtctgctgaggatacactgcaggctcagggtgaaatcagcaatgatgtggaagtggtcaaggaccagtttcacacccatgagggctacatgatggacctgacagcccaccagggcagagtgggaaatatcctgcagctgggctccaagctgattggcacaggcaagctgtctgaggatgaagagacagaggtgcaagagcagatgaacctgctgaacagcagatgggagtgtctgagagtggccagcatggaaaagcagagcaacctgcacagagtgctcatggacctgcagaatcagaaactgaaagaactgaatgactggctgaccaagacagaagaaaggactaggaagatggaagaggaacctctgggaccagacctggaagatctgaaaagacaggtgcagcagcataaggtgctgcaagaggaccttgagcaagagcaagtcagagtgaacagcctgacacacatggtggtggttgtggatgagtcctctggggatcatgccacagctgctctggaagaacagctgaaggtgctgggagacagatgggccaacatctgtaggtggacagaggatagatgggtgctgctccaggacattctgctgaagtggcagagactgacagaggaacagtgcctgttttctgcctggctctctgagaaagaggatgctgtcaacaagatccataccacaggcttcaaggatcagaatgagatgctcagctccctgcagaaactggctgtgctgaaggctgacctggaaaagaaaaagcagtccatgggcaagctctacagcctgaagcaggacctgctgtctaccctgaagaacaagtctgtgacccagaaaactgaggcctggctggacaactttgctagatgctgggacaacctggtgcagaagctggaaaagtctacagcccagatcagccagcaacctgatcttgcccctggcctgaccacaattggagcctctccaacacagactgtgaccctggttacccagccagtggtcaccaaagagacagccatcagcaaactggaaatgcccagctctctgatgctggaagtccccacactggaaaggctgcaagaacttcaagaggccacagatgagctggacctgaagctgagacaggctgaagtgatcaaaggcagctggcagccagttggggacctgctcattgatagcctgcaggaccatctggaaaaagtgaaagccctgaggggagagattgcccctctgaaagaaaatgtgtcccatgtgaatgacctggccagacagctgaccacactgggaatccagctgagcccctacaacctgagcacccttgaggacctgaacaccaggtggaagctcctccaggtggcagtggaagatagagtcaggcagctgcatgaggcccacagagattttggaccagccagccagcactttctgtctacctctgtgcaaggcccctgggagagagctatctctcctaacaaggtgccctactacatcaaccatgagacacagaccacctgttgggatcaccccaagatgacagagctgtaccagagtctggcagacctcaacaatgtcagattcagtgcctacaggactgccatgaagctcagaaggctccagaaagctctgtgcctggacctgctttccctgagtgcagcttgtgatgccctggaccagcacaatctgaagcagaatgaccagcctatggacatcctccagatcatcaactgcctcaccaccatctatgataggctggaacaagagcacaacaatctggtcaatgtgcccctgtgtgtggacatgtgcctgaattggctgctgaatgtgtatgacacaggcagaacaggcaggatcagagtcctgtccttcaagacaggcatcatctccctgtgcaaagcccacttggaggacaagtacagatacctgttcaagcaagtggcctccagcacaggcttttgtgaccagagaaggctgggcctgctcctgcatgacagcattcagatccctagacagctgggagaagtggcttcctttggaggcagcaatattgagccatcagtcaggtcctgttttcagtttgccaacaacaagcctgagattgaggctgccctgttcctggactggatgagacttgagcctcagagcatggtctggctgcctgtgcttcatagagtggctgctgctgagactgccaagcaccaggccaagtgcaacatctgcaaagagtgccccatcattggcttcagatacagatccctgaagcacttcaactatgatatctgccagagctgcttctttagtggcagggttgccaagggccacaaaatgcactaccccatggtggaatactgcaccccaacaacctctggggaagatgttagagactttgccaaggtgctgaaaaacaagttcaggaccaagagatactttgctaagcaccccagaatgggctacctgcctgtccagacagtgcttgagggtgacaacatggaaacccctgtgacactgatcaatttctggccagtggactctgcccctgcctcaagtccacagctgtcccatgatgacacccacagcagaattgagcactatgcctccagactggcagagatggaaaacagcaatggcagctacctgaatgatagcatcagccccaatgagagcattgatgatgagcatctgctgatccagcactactgtcagtccctgaaccaggactctccactgagccagcctagaagccctgctcagatcctgatcagccttgagtctgaggaaaggggagagctggaaagaatcctggcagatcttgaggaagagaacagaaacctgcaggcagagtatgacaggctcaaacagcagcatgagcacaagggactgagccctctgccttctcctcctgaaatgatgcccacctctccacagtctccaaggtgatga

SEQ ID NO: 39 - DNA, 4734 bp, synthetic construct
  source 1..4734: mol_type = other DNA
ctgcgcgctcgctcgctcactgaggccgcccgggcaaagcccgggcgtcgggcgacctttggtcgcccggcctcagtgagcgagcgagcgcgcagagagggagtggccaactccatcactaggggttcctcatatgcagggtaatggggatcctctagaggccgtccgccctcggcaccatcctcacgacacccaaatatggcgacgggtgaggaatggtggggagttatttttagagcggtgaggaaggtgggcaggcagcaggtgttggcgctccatatttggcgggagttatttttagagcggaggaatggtggacacccaaatatggcgacggttcctcacccgtcgctaaaaataactccgtgtccgccctcggccggggccgcattcctgggggccgggcggtgctcccgcccgcctcgataaaaggctccggggccggcggcggcccacgagctacccggaggagcgggaggcgccaagcggaattcgccaccatgctttggtgggaagaggtggaagattgctatgagagggaagatgtgcagaagaaaaccttcaccaaatgggtcaatgcccagttcagcaagtttggcaagcagcacattgagaacctgttcagtgacctgcaggatggcagaaggctgctggatctgctggaaggcctgacaggccagaagctgcctaaagagaagggcagcacaagagtgcatgccctgaacaatgtgaacaaggccctgagagtgctgcagaacaacaatgtggacctggtcaatattggcagcacagacattgtggatggcaaccacaagctgaccctgggcctgatctggaacatcatcctgcactggcaagtgaagaatgtgatgaagaacatcatggctggcctgcagcagaccaactctgagaagatcctgctgagctgggtcagacagagcaccagaaactaccctcaagtgaatgtgatcaacttcaccacctcttggagtgatggactggccctgaatgccctgatccacagccacagacctgacctgtttgactggaactctgttgtgtgccagcagtctgccacacagagactggaacatgccttcaacattgccagataccagctgggaattgagaaactgctggaccctgaggatgtggacaccacctatcctgacaagaaatccatcctcatgtacatcaccagcctgttccaggtgctgccccagcaagtgtccattgaggccattcaagaggttgagatgctgcccagacctcctaaagtgaccaaagaggaacacttccagctgcaccaccagatgcactactctcagcagatcacagtgtctctggcccagggatatgagagaacaagcagccccaagcctaggttcaagagctatgcctacacacaggctgcctatgtgaccacatctgaccccacaagaagcccatttccaagccagcatctggaagcccctgaggacaagagctttggcagcagcctgatggaatctgaagtgaacctggatagataccagacagccctggaagaagtgctgtcctggctgctgtctgctgaggatacactgcaggctcagggtgaaatcagcaatgatgtggaagtggtcaaggaccagtttcacacccatgagggctacatgatggacctgacagcccaccagggcagagtgggaaatatcctgcagctgggctccaagctgattggcacaggcaagctgtctgaggatgaagagacagaggtgcaagagcagatgaacctgctgaacagcagatgggagtgtctgagagtggccagcatggaaaagcagagcaacctgcacagagtgctcatggacctgcagaatcagaaactgaaagaactgaatgactggctgaccaagacagaagaaaggactaggaagatggaagaggaacctctgggaccagacctggaagatctgaaaagacaggtgcagcagcataaggtgctgcaagaggaccttgagcaagagcaagtcagagtgaacagcctgacacacatggtggtggttgtggatgagtcctctggggatcatgccacagctgctctggaagaacagctgaaggtgctgggagacagatgggccaacatctgtaggtggacagaggatagatgggtgctgctccaggacattctgctgaagtggcagagactgacagaggaacagtgcctgttttctgcctggctctctgagaaagaggatgctgtcaacaagatccataccacaggcttcaaggatcagaatgagatgctcagctccctgcagaaactggctgtgctgaaggctgacctggaaaagaaaaagcagtccatgggcaagctctacagcctgaagcaggacctgctgtctaccctgaagaacaagtctgtgacccagaaaactgaggcctggctggacaactttgctagatgctgggacaacctggtgcagaagctggaaaagtctacagcccagatcagccagcaacctgatcttgcccctggcctgaccacaattggagcctctccaacacagactgtgaccctggttacccagccagtggtcaccaaagagacagccatcagcaaactggaaatgcccagctctctgatgctggaagtccccacactggaaaggctgcaagaacttcaagaggccacagatgagctggacctgaagctgagacaggctgaagtgatcaaaggcagctggcagccagttggggacctgctcattgatagcctgcaggaccatctggaaaaagtgaaagccctgaggggagagattgcccctctgaaagaaaatgtgtcccatgtgaatgacctggccagacagctgaccacactgggaatccagctgagcccctacaacctgagcacccttgaggacctgaacaccaggtggaagctcctccaggtggcagtggaagatagagtcaggcagctgcatgaggcccacagagattttggaccagccagccagcactttctgtctacctctgtgcaaggcccctgggagagagctatctctcctaacaaggtgccctactacatcaaccatgagacacagaccacctgttgggatcaccccaagatgacagagctgtaccagagtctggcagacctcaacaatgtcagattcagtgcctacaggactgccatgaagctcagaaggctccagaaagctctgtgcctggacctgctttccctgagtgcagcttgtgatgccctggaccagcacaatctgaagcagaatgaccagcctatggacatcctccagatcatcaactgcctcaccaccatctatgataggctggaacaagagcacaacaatctggtcaatgtgcccctgtgtgtggacatgtgcctgaattggctgctgaatgtgtatgacacaggcagaacaggcaggatcagagtcctgtccttcaagacaggcatcatctccctgtgcaaagcccacttggaggacaagtacagatacctgttcaagcaagtggcctccagcacaggcttttgtgaccagagaaggctgggcctgctcctgcatgacagcattcagatccctagacagctgggagaagtggcttcctttggaggcagcaatattgagccatcagtcaggtcctgttttcagtttgccaacaacaagcctgagattgaggctgccctgttcctggactggatgagacttgagcctcagagcatggtctggctgcctgtgcttcatagagtggctgctgctgagactgccaagcaccaggccaagtgcaacatctgcaaagagtgccccatcattggcttcagatacagatccctgaagcacttcaactatgatatctgccagagctgcttctttagtggcagggttgccaagggccacaaaatgcactaccccatggtggaatactgcaccccaacaacctctggggaagatgttagagactttgccaaggtgctgaaaaacaagttcaggaccaagagatactttgctaagcaccccagaatgggctacctgcctgtccagacagtgcttgagggtgacaacatggaaacccctgtgacactgatcaatttctggccagtggactctgcccctgcctcaagtccacagctgtcccatgatgacacccacagcagaattgagcactatgcctccagactggcagagatggaaaacagcaatggcagctacctgaatgatagcatcagccccaatgagagcattgatgatgagcatctgctgatccagcactactgtcagtccctgaaccaggactctccactgagccagcctagaagccctgctcagatcctgatcagccttgagtctgaggaaaggggagagctggaaagaatcctggcagatcttgaggaagagaacagaaacctgcaggcagagtatgacaggctcaaacagcagcatgagcacaagggactgagccctctgccttctcctcctgaaatgatgcccacctctccacagtctccaaggtgatgactcgagaggcctaataaagagctcagatgcatcgatcagagtgtgttggttttttgtgtgccagggtaatgggctagctgcggccgcaggaacccctagtgatggagttggccactccctctctgcgcgctcgctcgctcactgaggccgggcgaccaaaggtcgcccgacgcccgggctttgcccgggcggcctcagtgagcgagcgagcgcgcag

SEQ ID NO: 40 - DNA, 3920 bp, synthetic construct
  source 1..3920: mol_type = other DNA
ggccgtccgccctcggcaccatcctcacgacacccaaatatggcgacgggtgaggaatggtggggagttatttttagagcggtgaggaaggtgggcaggcagcaggtgttgggggagttatttttagagcggggagttatttttagagcggaggaatggtggacacccaaatatggcgacggttcctcacggacacccaaatatggcgacgggccctcggccggggccgcattcctgggggccgggcggtgctcccgcccgcctcgataaaaggctccggggccggcggcggcccacgagctacccggaggagcgggaggcgccaagcggaattcgccaccatgctttggtgggaagaggtggaagattgctatgagagggaagatgtgcagaagaaaaccttcaccaaatgggtcaatgcccagttcagcaagtttggcaagcagcacattgagaacctgttcagtgacctgcaggatggcagaaggctgctggatctgctggaaggcctgacaggccagaagctgcctaaagagaagggcagcacaagagtgcatgccctgaacaatgtgaacaaggccctgagagtgctgcagaacaacaatgtggacctggtcaatattggcagcacagacattgtggatggcaaccacaagctgaccctgggcctgatctggaacatcatcctgcactggcaagtgaagaatgtgatgaagaacatcatggctggcctgcagcagaccaactctgagaagatcctgctgagctgggtcagacagagcaccagaaactaccctcaagtgaatgtgatcaacttcaccacctcttggagtgatggactggccctgaatgccctgatccacagccacagacctgacctgtttgactggaactctgttgtgtgccagcagtctgccacacagagactggaacatgccttcaacattgccagataccagctgggaattgagaaactgctggaccctgaggatgtggacaccacctatcctgacaagaaatccatcctcatgtacatcaccagcctgttccaggtgctgccccagcaagtgtccattgaggccattcaagaggttgagatgctgcccagacctcctaaagtgaccaaagaggaacacttccagctgcaccaccagatgcactactctcagcagatcacagtgtctctggcccagggatatgagagaacaagcagccccaagcctaggttcaagagctatgcctacacacaggctgcctatgtgaccacatctgaccccacaagaagcccatttccaagccagcatctggaagcccctgaggacaagagctttggcagcagcctgatggaatctgaagtgaacctggatagataccagacagccctggaagaagtgctgtcctggctgctgtctgctgaggatacactgcaggctcagggtgaaatcagcaatgatgtggaagtggtcaaggaccagtttcacacccatgagggctacatgatggacctgacagcccaccagggcagagtgggaaatatcctgcagctgggctccaagctgattggcacaggcaagctgtctgaggatgaagagacagaggtgcaagagcagatgaacctgctgaacagcagatgggagtgtctgagagtggccagcatggaaaagcagagcaacctgcacagagtgctcatggacctgcagaatcagaaactgaaagaactgaatgactggctgaccaagacagaagaaaggactaggaagatggaagaggaacctctgggaccagacctggaagatctgaaaagacaggtgcagcagcataaggtgctgcaagaggaccttgagcaagagcaagtcagagtgaacagcctgacacacatggtggtggttgtggatgagtcctctggggatcatgccacagctgctctggaagaacagctgaaggtgctgggagacagatgggccaacatctgtaggtggacagaggatagatgggtgctgctccaggacattctgctgaagtggcagagactgacagaggaacagtgcctgttttctgcctggctctctgagaaagaggatgctgtcaacaagatccataccacaggcttcaaggatcagaatgagatgctcagctccctgcagaaactggctgtgctgaaggctgacctggaaaagaaaaagcagtccatgggcaagctctacagcctgaagcaggacctgctgtctaccctgaagaacaagtctgtgacccagaaaactgaggcctggctggacaactttgctagatgctgggacaacctggtgcagaagctggaaaagtctacagcccagatcagccagcaacctgatcttgcccctggcctgaccacaattggagcctctccaacacagactgtgaccctggttacccagccagtggtcaccaaagagacagccatcagcaaactggaaatgcccagctctctgatgctggaagtccccacactggaaaggctgcaagaacttcaagaggccacagatgagctggacctgaagctgagacaggctgaagtgatcaaaggcagctggcagccagttggggacctgctcattgatagcctgcaggaccatctggaaaaagtgaaagccctgaggggagagattgcccctctgaaagaaaatgtgtcccatgtgaatgacctggccagacagctgaccacactgggaatccagctgagcccctacaacctgagcacccttgaggacctgaacaccaggtggaagctcctccaggtggcagtggaagatagagtcaggcagctgcatgaggcccacagagattttggaccagccagccagcactttctgtctacctctgtgcaaggcccctgggagagagctatctctcctaacaaggtgccctactacatcaaccatgagacacagaccacctgttgggatcaccccaagatgacagagctgtaccagagtctggcagacctcaacaatgtcagattcagtgcctacaggactgccatgaagctcagaaggctccagaaagctctgtgcctggacctgctttccctgagtgcagcttgtgatgccctggaccagcacaatctgaagcagaatgaccagcctatggacatcctccagatcatcaactgcctcaccaccatctatgataggctggaacaagagcacaacaatctggtcaatgtgcccctgtgtgtggacatgtgcctgaattggctgctgaatgtgtatgacacaggcagaacaggcaggatcagagtcctgtccttcaagacaggcatcatctccctgtgcaaagcccacttggaggacaagtacagatacctgttcaagcaagtggcctccagcacaggcttttgtgaccagagaaggctgggcctgctcctgcatgacagcattcagatccctagacagctgggagaagtggcttcctttggaggcagcaatattgagccatcagtcaggtcctgttttcagtttgccaacaacaagcctgagattgaggctgccctgttcctggactggatgagacttgagcctcagagcatggtctggctgcctgtgcttcatagagtggctgctgctgagactgccaagcaccaggccaagtgcaacatctgcaaagagtgccccatcattggcttcagatacagatccctgaagcacttcaactatgatatctgccagagctgcttctttagtggcagggttgccaagggccacaaaatgcactaccccatggtggaatactgcaccccaacaacctctggggaagatgttagagactttgccaaggtgctgaaaaacaagttcaggaccaagagatactttgctaagcaccccagaatgggctacctgcctgtccagacagtgcttgagggtgacaacatggaaacctgatga

SEQ ID NO: 41 - DNA, 4284 bp, synthetic construct
  source 1..4284: mol_type = other DNA
ctgcgcgctcgctcgctcactgaggccgcccgggcaaagcccgggcgtcgggcgacctttggtcgcccggcctcagtgagcgagcgagcgcgcagagagggagtggccaactccatcactaggggttcctcatatgcagggtaatggggatcctctagaggccgtccgccctcggcaccatcctcacgacacccaaatatggcgacgggtgaggaatggtggggagttatttttagagcggtgaggaaggtgggcaggcagcaggtgttgggggagttatttttagagcggggagttatttttagagcggaggaatggtggacacccaaatatggcgacggttcctcacggacacccaaatatggcgacgggccctcggccggggccgcattcctgggggccgggcggtgctcccgcccgcctcgataaaaggctccggggccggcggcggcccacgagctacccggaggagcgggaggcgccaagcggaattcgccaccatgctttggtgggaagaggtggaagattgctatgagagggaagatgtgcagaagaaaaccttcaccaaatgggtcaatgcccagttcagcaagtttggcaagcagcacattgagaacctgttcagtgacctgcaggatggcagaaggctgctggatctgctggaaggcctgacaggccagaagctgcctaaagagaagggcagcacaagagtgcatgccctgaacaatgtgaacaaggccctgagagtgctgcagaacaacaatgtggacctggtcaatattggcagcacagacattgtggatggcaaccacaagctgaccctgggcctgatctggaacatcatcctgcactggcaagtgaagaatgtgatgaagaacatcatggctggcctgcagcagaccaactctgagaagatcctgctgagctgggtcagacagagcaccagaaactaccctcaagtgaatgtgatcaacttcaccacctcttggagtgatggactggccctgaatgccctgatccacagccacagacctgacctgtttgactggaactctgttgtgtgccagcagtctgccacacagagactggaacatgccttcaacattgccagataccagctgggaattgagaaactgctggaccctgaggatgtggacaccacctatcctgacaagaaatccatcctcatgtacatcaccagcctgttccaggtgctgccccagcaagtgtccattgaggccattcaagaggttgagatgctgcccagacctcctaaagtgaccaaagaggaacacttccagctgcaccaccagatgcactactctcagcagatcacagtgtctctggcccagggatatgagagaacaagcagccccaagcctaggttcaagagctatgcctacacacaggctgcctatgtgaccacatctgaccccacaagaagcccatttccaagccagcatctggaagcccctgaggacaagagctttggcagcagcctgatggaatctgaagtgaacctggatagataccagacagccctggaagaagtgctgtcctggctgctgtctgctgaggatacactgcaggctcagggtgaaatcagcaatgatgtggaagtggtcaaggaccagtttcacacccatgagggctacatgatggacctgacagcccaccagggcagagtgggaaatatcctgcagctgggctccaagctgattggcacaggcaagctgtctgaggatgaagagacagaggtgcaagagcagatgaacctgctgaacagcagatgggagtgtctgagagtggccagcatggaaaagcagagcaacctgcacagagtgctcatggacctgcagaatcagaaactgaaagaactgaatgactggctgaccaagacagaagaaaggactaggaagatggaagaggaacctctgggaccagacctggaagatctgaaaagacaggtgcagcagcataaggtgctgcaagaggaccttgagcaagagcaagtcagagtgaacagcctgacacacatggtggtggttgtggatgagtcctctggggatcatgccacagctgctctggaagaacagctgaaggtgctgggagacagatgggccaacatctgtaggtggacagaggatagatgggtgctgctccaggacattctgctgaagtggcagagactgacagaggaacagtgcctgttttctgcctggctctctgagaaagaggatgctgtcaacaagatccataccacaggcttcaaggatcagaatgagatgctcagctccctgcagaaactggctgtgctgaaggctgacctggaaaagaaaaagcagtccatgggcaagctctacagcctgaagcaggacctgctgtctaccctgaagaacaagtctgtgacccagaaaactgaggcctggctggacaactttgctagatgctgggacaacctggtgcagaagctggaaaagtctacagcccagatcagccagcaacctgatcttgcccctggcctgaccacaattggagcctctccaacacagactgtgaccctggttacccagccagtggtcaccaaagagacagccatcagcaaactggaaatgcccagctctctgatgctggaagtccccacactggaaaggctgcaagaacttcaagaggccacagatgagctggacctgaagctgagacaggctgaagtgatcaaaggcagctggcagccagttggggacctgctcattgatagcctgcaggaccatctggaaaaagtgaaagccctgaggggagagattgcccctctgaaagaaaatgtgtcccatgtgaatgacctggccagacagctgaccacactgggaatccagctgagcccctacaacctgagcacccttgaggacctgaacaccaggtggaagctcctccaggtggcagtggaagatagagtcaggcagctgcatgaggcccacagagattttggaccagccagccagcactttctgtctacctctgtgcaaggcccctgggagagagctatctctcctaacaaggtgccctactacatcaaccatgagacacagaccacctgttgggatcaccccaagatgacagagctgtaccagagtctggcagacctcaacaatgtcagattcagtgcctacaggactgccatgaagctcagaaggctccagaaagctctgtgcctggacctgctttccctgagtgcagcttgtgatgccctggaccagcacaatctgaagcagaatgaccagcctatggacatcctccagatcatcaactgcctcaccaccatctatgataggctggaacaagagcacaacaatctggtcaatgtgcccctgtgtgtggacatgtgcctgaattggctgctgaatgtgtatgacacaggcagaacaggcaggatcagagtcctgtccttcaagacaggcatcatctccctgtgcaaagcccacttggaggacaagtacagatacctgttcaagcaagtggcctccagcacaggcttttgtgaccagagaaggctgggcctgctcctgcatgacagcattcagatccctagacagctgggagaagtggcttcctttggaggcagcaatattgagccatcagtcaggtcctgttttcagtttgccaacaacaagcctgagattgaggctgccctgttcctggactggatgagacttgagcctcagagcatggtctggctgcctgtgcttcatagagtggctgctgctgagactgccaagcaccaggccaagtgcaacatctgcaaagagtgccccatcattggcttcagatacagatccctgaagcacttcaactatgatatctgccagagctgcttctttagtggcagggttgccaagggccacaaaatgcactaccccatggtggaatactgcaccccaacaacctctggggaagatgttagagactttgccaaggtgctgaaaaacaagttcaggaccaagagatactttgctaagcaccccagaatgggctacctgcctgtccagacagtgcttgagggtgacaacatggaaacctgatgagtcgacaggcctaataaagagctcagatgcatcgatcagagtgtgttggttttttgtgtggctagctgcggccgcaggaacccctagtgatggagttggccactccctctctgcgcgctcgctcgctcactgaggccgggcgaccaaaggtcgcccgacgcccgggctttgcccgggcggcctcagtgagcgagcgagcgcgcag

SEQ ID NO: 42 - protein, 7 aa, synthetic construct
LGETTRP

SEQ ID NO: 43 - protein, 9 aa, synthetic construct
LALGETTRP

SEQ ID NO: 44 - DNA, 100 bp, synthetic construct
  source 1..100: mol_type = other DNA
aggttaatttttaaaaagcagtcaaaagtccaagtggcccttggcagcatttactctctctgtttgctctggttaataatctcaggagcacaaacattcc

SEQ ID NO: 45 - DNA, 200 bp, synthetic construct
  source 1..200: mol_type = other DNA
aggttaatttttaaaaagcagtcaaaagtccaagtggcccttggcagcatttactctctctgtttgctctggttaataatctcaggagcacaaacattccaggttaatttttaaaaagcagtcaaaagtccaagtggcccttggcagcatttactctctctgtttgctctggttaataatctcaggagcacaaacattcc

SEQ ID NO: 46 - DNA, 321 bp, synthetic construct
  source 1..321: mol_type = other DNA
aggctcagaggcacacaggagtttctgggctcaccctgcccccttccaacccctcagttcccatcctccagcagctgtttgtgtgctgcctctgaagtccacactgaacaaacttcagcctactcatgtccctaaaatgggcaaacattgcaagcagcaaacagcaaacacacagccctccctgcctgctgaccttggagctggggcagaggtcagagacctctctgggcccatgccacctccaacatccactcgaccccttggaatttcggtggagaggagcagaggttgtcctggcgtggtttaggtagtgtgagaggg

SEQ ID NO: 47 - DNA, 554 bp, synthetic construct
  source 1..554: mol_type = other DNA
aggctcagaggcacacaggagtttctgggctcaccctgcccccttccaacccctcagttcccatcctccagcagctgtttgtgtgctgcctctgaagtccacactgaacaaacttcagcctactcatgtccctaaaatgggcaaacattgcaagcagcaaacagcaaacacacagccctccctgcctgctgaccttggagctggggcagaggtcagagacctctctgggcccatgccacctccaacatccactcgaccccttggaatttcggtggagaggagcagaggttgtcctggcgtggtttaggtagtgtgagagggtctagaaggctcagaggcacacaggagtttctgggctcaccctgcccccttccaacccctcagttcccatcctccagcagctgtttgtgtgctgcctctgaagtccacactgaacaaacttcagcctactcatgtccctaaaatgggcaaacattgcaagcagcaaacagcaaacacacagccctccctgcctgctgaccttggagctggggcagaggtcagagacctctctg

SEQ ID NO: 48 - DNA, 460 bp, synthetic construct
  source 1..460: mol_type = other DNA
gggctggaagctacctttgacatcatttcctctgcgaatgcatgtataatttctacagaacctattagaaaggatcacccagcctctgcttttgtacaactttcccttaaaaaactgccaattccactgctgtttggcccaatagtgagaactttttcctgctgcctcttggtgcttttgcctatggcccctattctgcctgctgaagacactcttgccagcatggacttaaacccctccagctctgacaatcctctttctcttttgttttacatgaagggtctggcagccaaagcaatcactcaaagttcaaaccttatcattttttgctttgttcctcttggccttggttttgtacatcagctttgaaaataccatcccagggttaatgctggggttaatttataactaagagtgctctagttttgcaatacaggacatgctataaaaatggaaagat

SEQ ID NO: 49 - DNA, 393 bp, synthetic construct
  source 1..393: mol_type = other DNA
gatcttgctaccagtggaacagccactaaggattctgcagtgagagcagagggccagctaagtggtactctcccagagactgtctgactcacgccaccccctccaccttggacacaggacgctgtggtttctgagccaggtacaatgactcctttcggtaagtgcagtggaagctgtacactgcccaggcaaagcgtccgggcagcgtaggcgggcgactcagatcccagccagtggacttagcccctgtttgctcctccgataactggggtgaccttggttaatattcaccagcagcctcccccgttgcccctctggatccactgcttaaatacggacgaggacagggccctgtctcctcagcttcaggcaccaccactgacctgggacagt

SEQ ID NO: 50 - DNA, 393 bp, synthetic construct
  source 1..393: mol_type = other DNA
gatcttgctaccagtggaacagccactaaggattctgcagtgagagcagagggccagctaagtggtactctcccagagactgtctgactcacgccaccccctccaccttggacacaggacgctgtggtttctgagccaggtacagtgactcctttcggtaagtgcagtggaagctgtacactgcccaggcaaagcgtccgggcagcgtaggcgggcgactcagatcccagccagtggacttagcccctgtttgctcctccgataactggggtgaccttggttaatattcaccagcagcctcccccgttgcccctctggatccactgcttaaatacggacgaggacagggccctgtctcctcagcttcaggcaccaccactgacctgggacagt

SEQ ID NO: 51 - DNA, 723 bp, synthetic construct
  source 1..723: mol_type = other DNA
aggctcagaggcacacaggagtttctgggctcaccctgcccccttccaacccctcagttcccatcctccagcagctgtttgtgtgctgcctctgaagtccacactgaacaaacttcagcctactcatgtccctaaaatgggcaaacattgcaagcagcaaacagcaaacacacagccctccctgcctgctgaccttggagctggggcagaggtcagagacctctctgggcccatgccacctccaacatccactcgaccccttggaatttcggtggagaggagcagaggttgtcctggcgtggtttaggtagtgtgagaggggtacccggggatcttgctaccagtggaacagccactaaggattctgcagtgagagcagagggccagctaagtggtactctcccagagactgtctgactcacgccaccccctccaccttggacacaggacgctgtggtttctgagccaggtacaatgactcctttcggtaagtgcagtggaagctgtacactgcccaggcaaagcgtccgggcagcgtaggcgggcgactcagatcccagccagtggacttagcccctgtttgctcctccgataactggggtgaccttggttaatattcaccagcagcctcccccgttgcccctctggatccactgcttaaatacggacgaggacagggccctgtctcctcagcttcaggcaccaccactgacctgggacagt

SEQ ID NO: 52 - DNA, 433 bp, synthetic construct
  source 1..433: mol_type = other DNA
ccctgcatgcgaagatcttcgaacaaggctgtgggggactgagggcaggctgtaacaggcttgggggccagggcttatacgtgcctgggactcccaaagtattactgttccatgttcccggcgaagggccagctgtcccccgccagctagactcagcacttagtttaggaaccagtgagcaagtcagcccttggggcagcccatacaaggccatggggctgggcaagctgcacgcctgggtccggggtgggcacggtgcccgggcaacgagctgaaagctcatctgctctcaggggcccctccctggggacagcccctcctggctagtcacaccctgtaggctcctctatataacccaggggcacaggggctgccctcattctaccaccacctccacagcacagacagacactcaggagccagccagcgtcga

SEQ ID NO: 53 - DNA, 770 bp, synthetic construct
  source 1..770: mol_type = other DNA
ctagaagctgcatgtctaagctagacccttcagattaaaaataactgaggtaagggcctgggtaggggaggtggtgtgagacgctcctgtctctcctctatctgcccatcggccctttggggaggaggaatgtgcccaaggactaaaaaaaggccatggagccagaggggcgagggcaacagacctttcatgggcaaaccttggggccctgctgtctagcatgccccactacgggtctaggctgcccatgtaaggaggcaaggcctggggacacccgagatgcctggttataattaacccagacatgtggctgcccccccccccccaacacctgctgcctctaaaaataaccctgtccctggtggatcccctgcatgcgaagatcttcgaacaaggctgtgggggactgagggcaggctgtaacaggcttgggggccagggcttatacgtgcctgggactcccaaagtattactgttccatgttcccggcgaagggccagctgtcccccgccagctagactcagcacttagtttaggaaccagtgagcaagtcagcccttggggcagcccatacaaggccatggggctgggcaagctgcacgcctgggtccggggtgggcacggtgcccgggcaacgagctgaaagctcatctgctctcaggggcccctccctggggacagcccctcctggctagtcacaccctgtaggctcctctatataacccaggggcacaggggctgccctcattctaccaccacctccacagcac

SEQ ID NO: 54 - DNA, 400 bp, synthetic construct
  source 1..400: mol_type = other DNA
cggccgtccgccctcggcaccattcctcacgacaccgaaatatggcgacgggtgaggaatggtggggagttatttttagagcggtgaggaatggtgggcaggcagcaggtgttgggggagttatttttagagcggggagttatttttagagcggtgaggaatggtggacaccgaaatatggcgacgggtgaggaatggtgccgtcgccatatttgggtgtcccgtccgccctcggccggggccgcattcctgggggccgggcggtgctcccgcccgcctcgataaaaggctccggggccggcggcggcccacgagctacccggaggagcgggaggcgtctctgccagcggtccgacgcgcagtcagcaccaggtaggtgggcaccgcgccgtgccgtgcc

SEQ ID NO: 55 - DNA, 577 bp, synthetic construct
  source 1..577: mol_type = other DNA
ccactacgggtttaggctgcccatgtaaggaggcaaggcctggggacacccgagatgcctggttataattaacccagacatgtggctgccccccccccccccaacacctgctgcctctaaaaataaccctgtccctggtggatcccctgcatgcgaagatcttcgaacaaggctgtgggggactgagggcaggctgtaacaggcttgggggccagggcttatacgtgcctgggactcccaaagtattactgttccatgttcccggcgaagggccagctgtcccccgccagctagactcagcacttagtttaggaaccagtgagcaagtcagcccttggggcagcccatacaaggccatggggctgggcaagctgcacgcctgggtccggggtgggcacggtgcccgggcaacgagctgaaagctcatctgctctcaggggcccctccctggggacagcccctcctggctagtcacaccctgtaggctcctctatataacccaggggcacaggggctgccctcattctaccaccacctccacagcacagacagacactcaggagccagccagcgtcga

SEQ ID NO: 56 - protein, 1197 aa, synthetic construct
MLWWEEVEDCYEREDVQKKTFTKWVNAQFSKFGKQHIENLFSDLQDGRRLLDLLEGLTGQKLPKEKGSTRVHALNNVNKALRVLQNNNVDLVNIGSTDIVDGNHKLTLGLIWNIILHWQVKNVMKNIMAGLQQTNSEKILLSWVRQSTRNYPQVNVINFTTSWSDGLALNALIHSHRPDLFDWNSVVCQQSATQRLEHAFNIARYQLGIEKLLDPEDVDTTYPDKKSILMYITSLFQVLPQQVSIEAIQEVEMLPRPPKVTKEEHFQLHHQMHYSQQITVSLAQGYERTSSPKPRFKSYAYTQAAYVTTSDPTRSPFPSQHLEAPEDKSFGSSLMESEVNLDRYQTALEEVLSWLLSAEDTLQAQGEISNDVEVVKDQFHTHEGYMMDLTAHQGRVGNILQLGSKLIGTGKLSEDEETEVQEQMNLLNSRWECLRVASMEKQSNLHRVLMDLQNQKLKELNDWLTKTEERTRKMEEEPLGPDLEDLKRQVQQHKVLQEDLEQEQVRVNSLTHMVVVVDESSGDHATAALEEQLKVLGDRWANICRWTEDRWVLLQDILLKWQRLTEEQCLFSAWLSEKEDAVNKIHTTGFKDQNEMLSSLQKLAVLKADLEKKKQSMGKLYSLKQDLLSTLKNKSVTQKTEAWLDNFARCWDNLVQKLEKSTAQISQAVTTTQPSLTQTTVMETVTTVTTREQILVKHAQEELPPPPPQKKRQITVDTLERLQELQEATDELDLKLRQAEVIKGSWQPVGDLLIDSLQDHLEKVKALRGEIAPLKENVSHVNDLARQLTTLGIQLSPYNLSTLEDLNTRWKLLQVAVEDRVRQLHEAHRDFGPASQHFLSTSVQGPWERAISPNKVPYYINHETQTTCWDHPKMTELYQSLADLNNVRFSAYRTAMKLRRLQKALCLDLLSLSAACDALDQHNLKQNDQPMDILQIINCLTTIYDRLEQEHNNLVNVPLCVDMCLNWLLNVYDTGRTGRIRVLSFKTGIISLCKAHLEDKYRYLFKQVASSTGFCDQRRLGLLLHDSIQIPRQLGEVASFGGSNIEPSVRSCFQFANNKPEIEAALFLDWMRLEPQSMVWLPVLHRVAAAETAKHQAKCNICKECPIIGFRYRSLKHFNYDICQSCFFSGRVAKGHKMHYPMVEYCTPTTSGEDVRDFAKVLKNKFRTKRYFAKHPRMGYLPVQTVLEGDNMETDTM

SEQ ID NO: 57 - protein, 1192 aa, Homo sapiens
MLWWEEVEDCYEREDVQKKTFTKWVNAQFSKFGKQHIENLFSDLQDGRRLLDLLEGLTGQKLPKEKGSTRVHALNNVNKALRVLQNNNVDLVNIGSTDIVDGNHKLTLGLIWNIILHWQVKNVMKNIMAGLQQTNSEKILLSWVRQSTRNYPQVNVINFTTSWSDGLALNALIHSHRPDLFDWNSVVCQQSATQRLEHAFNIARYQLGIEKLLDPEDVDTTYPDKKSILMYITSLFQVLPQQVSIEAIQEVEMLPRPPKVTKEEHFQLHHQMHYSQQITVSLAQGYERTSSPKPRFKSYAYTQAAYVTTSDPTRSPFPSQHLEAPEDKSFGSSLMESEVNLDRYQTALEEVLSWLLSAEDTLQAQGEISNDVEVVKDQFHTHEGYMMDLTAHQGRVGNILQLGSKLIGTGKLSEDEETEVQEQMNLLNSRWECLRVASMEKQSNLHRVLMDLQNQKLKELNDWLTKTEERTRKMEEEPLGPDLEDLKRQVQQHKVLQEDLEQEQVRVNSLTHMVVVVDESSGDHATAALEEQLKVLGDRWANICRWTEDRWVLLQDILLKWQRLTEEQCLFSAWLSEKEDAVNKIHTTGFKDQNEMLSSLQKLAVLKADLEKKKQSMGKLYSLKQDLLSTLKNKSVTQKTEAWLDNFARCWDNLVQKLEKSTAQISQAVTTTQPSLTQTTVMETVTTVTTREQILVKHAQEELPPPPPQKKRTLERLQELQEATDELDLKLRQAEVIKGSWQPVGDLLIDSLQDHLEKVKALRGEIAPLKENVSHVNDLARQLTTLGIQLSPYNLSTLEDLNTRWKLLQVAVEDRVRQLHEAHRDFGPASQHFLSTSVQGPWERAISPNKVPYYINHETQTTCWDHPKMTELYQSLADLNNVRFSAYRTAMKLRRLQKALCLDLLSLSAACDALDQHNLKQNDQPMDILQIINCLTTIYDRLEQEHNNLVNVPLCVDMCLNWLLNVYDTGRTGRIRVLSFKTGIISLCKAHLEDKYRYLFKQVASSTGFCDQRRLGLLLHDSIQIPRQLGEVASFGGSNIEPSVRSCFQFANNKPEIEAALFLDWMRLEPQSMVWLPVLHRVAAAETAKHQAKCNICKECPIIGFRYRSLKHFNYDICQSCFFSGRVAKGHKMHYPMVEYCTPTTSGEDVRDFAKVLKNKFRTKRYFAKHPRMGYLPVQTVLEGDNMETDTM

SEQ ID NO: 58 - protein, 1325 aa, synthetic construct
MLWWEEVEDCYEREDVQKKTFTKWVNAQFSKFGKQHIENLFSDLQDGRRLLDLLEGLTGQKLPKEKGSTRVHALNNVNKALRVLQNNNVDLVNIGSTDIVDGNHKLTLGLIWNIILHWQVKNVMKNIMAGLQQTNSEKILLSWVRQSTRNYPQVNVINFTTSWSDGLALNALIHSHRPDLFDWNSVVCQQSATQRLEHAFNIARYQLGIEKLLDPEDVDTTYPDKKSILMYITSLFQVLPQQVSIEAIQEVEMLPRPPKVTKEEHFQLHHQMHYSQQITVSLAQGYERTSSPKPRFKSYAYTQAAYVTTSDPTRSPFPSQHLEAPEDKSFGSSLMESEVNLDRYQTALEEVLSWLLSAEDTLQAQGEISNDVEVVKDQFHTHEGYMMDLTAHQGRVGNILQLGSKLIGTGKLSEDEETEVQEQMNLLNSRWECLRVASMEKQSNLHRVLMDLQNQKLKELNDWLTKTEERTRKMEEEPLGPDLEDLKRQVQQHKVLQEDLEQEQVRVNSLTHMVVVVDESSGDHATAALEEQLKVLGDRWANICRWTEDRWVLLQDQPDLAPGLTTIGASPTQTVTLVTQPVVTKETAISKLEMPSSLMLEVPTHRLLQQFPLDLEKFLAWLTEAETTANVLQDATRKERLLEDSKGVKELMKQWQDLQGEIEAHTDVYHNLDENSQKILRSLEGSDDAVLLQRRLDNMNFKWSELRKKSLNIRSHLEASSDQWKRLHLSLQELLVWLQLKDDELSRQAPIGGDFPAVQKQNDVHRAFKRELKTKEPVIMSTLETVRIFLTEQPLEGLEKLYQEPRELPPEERAQNVTRLLRKQAEEVNTEWEKLNLHSADWQRKIDETLERLQELQEATDELDLKLRQAEVIKGSWQPVGDLLIDSLQDHLEKVKALRGEIAPLKENVSHVNDLARQLTTLGIQLSPYNLSTLEDLNTRWKLLQVAVEDRVRQLHEAHRDFGPASQHFLSTSVQGPWERAISPNKVPYYINHETQTTCWDHPKMTELYQSLADLNNVRFSAYRTAMKLRRLQKALCLDLLSLSAACDALDQHNLKQNDQPMDILQIINCLTTIYDRLEQEHNNLVNVPLCVDMCLNWLLNVYDTGRTGRIRVLSFKTGIISLCKAHLEDKYRYLFKQVASSTGFCDQRRLGLLLHDSIQIPRQLGEVASFGGSNIEPSVRSCFQFANNKPEIEAALFLDWMRLEPQSMVWLPVLHRVAAAETAKHQAKCNICKECPIIGFRYRSLKHFNYDICQSCFFSGRVAKGHKMHYPMVEYCTPTTSGEDVRDFAKVLKNKFRTKRYFAKHPRMGYLPVQTVLEGDNMET

SEQ ID NO: 59 - protein, 1392 aa, Homo sapiens
MLWWEEVEDCYEREDVQKKTFTKWVNAQFSKFGKQHIENLFSDLQDGRRLLDLLEGLTGQKLPKEKGSTRVHALNNVNKALRVLQNNNVDLVNIGSTDIVDGNHKLTLGLIWNIILHWQVKNVMKNIMAGLQQTNSEKILLSWVRQSTRNYPQVNVINFTTSWSDGLALNALIHSHRPDLFDWNSVVCQQSATQRLEHAFNIARYQLGIEKLLDPEDVDTTYPDKKSILMYITSLFQVLPQQVSIEAIQEVEMLPRPPKVTKEEHFQLHHQMHYSQQITVSLAQGYERTSSPKPRFKSYAYTQAAYVTTSDPTRSPFPSQHLEAPEDKSFGSSLMESEVNLDRYQTALEEVLSWLLSAEDTLQAQGEISNDVEVVKDQFHTHEGYMMDLTAHQGRVGNILQLGSKLIGTGKLSEDEETEVQEQMNLLNSRWECLRVASMEKQSNLHRVLMDLQNQKLKELNDWLTKTEERTRKMEEEPLGPDLEDLKRQVQQHKVLQEDLEQEQVRVNSLTHMVVVVDESSGDHATAALEEQLKVLGDRWANICRWTEDRWVLLQDILLKWQRLTEEQCLFSAWLSEKEDAVNKIHTTGFKDQNEMLSSLQKLAVLKADLEKKKQSMGKLYSLKQDLLSTLKNKSVTQKTEAWLDNFARCWDNLVQKLEKSTAQISQAVTTTQPSLTQTTVMETVTTVTTREQILVKHAQEELPPPPPQKKRQITVDTLERLQELQEATDELDLKLRQAEVIKGSWQPVGDLLIDSLQDHLEKVKALRGEIAPLKENVSHVNDLARQLTTLGIQLSPYNLSTLEDLNTRWKLLQVAVEDRVRQLHEAHRDFGPASQHFLSTSVQGPWERAISPNKVPYYINHETQTTCWDHPKMTELYQSLADLNNVRFSAYRTAMKLRRLQKALCLDLLSLSAACDALDQHNLKQNDQPMDILQIINCLTTIYDRLEQEHNNLVNVPLCVDMCLNWLLNVYDTGRTGRIRVLSFKTGIISLCKAHLEDKYRYLFKQVASSTGFCDQRRLGLLLHDSIQIPRQLGEVASFGGSNIEPSVRSCFQFANNKPEIEAALFLDWMRLEPQSMVWLPVLHRVAAAETAKHQAKCNICKECPIIGFRYRSLKHFNYDICQSCFFSGRVAKGHKMHYPMVEYCTPTTSGEDVRDFAKVLKNKFRTKRYFAKHPRMGYLPVQTVLEGDNMETPVTLINFWPVDSAPASSPQLSHDDTHSRIEHYASRLAEMENSNGSYLNDSISPNESIDDEHLLIQHYCQSLNQDSPLSQPRSPAQILISLESEERGELERILADLEEENRNLQAEYDRLKQQHEHKGLSPLPSPPEMMPTSPQSPRDAELIAEAKLLRQHKGRLEARMQILEDHNKQLESQLHRLRQLLEQPQAEDTM

SEQ ID NO: 60 - protein, 1471 aa, Homo sapiens
MLWWEEVEDCYEREDVQKKTFTKWVNAQFSKFGKQHIENLFSDLQDGRRLLDLLEGLTGQKLPKEKGSTRVHALNNVNKALRVLQNNNVDLVNIGSTDIVDGNHKLTLGLIWNIILHWQVKNVMKNIMAGLQQTNSEKILLSWVRQSTRNYPQVNVINFTTSWSDGLALNALIHSHRPDLFDWNSVVCQQSATQRLEHAFNIARYQLGIEKLLDPEDVDTTYPDKKSILMYITSLFQVLPQQVSIEAIQEVEMLPRPPKVTKEEHFQLHHQMHYSQQITVSLAQGYERTSSPKPRFKSYAYTQAAYVTTSDPTRSPFPSQHLEAPEDKSFGSSLMESEVNLDRYQTALEEVLSWLLSAEDTLQAQGEISNDVEVVKDQFHTHEGYMMDLTAHQGRVGNILQLGSKLIGTGKLSEDEETEVQEQMNLLNSRWECLRVASMEKQSNLHRVLMDLQNQKLKELNDWLTKTEERTRKMEEEPLGPDLEDLKRQVQQHKVLQEDLEQEQVRVNSLTHMVVVVDESSGDHATAALEEQLKVLGDRWANICRWTEDRWVLLQDILLKWQRLTEEQCLFSAWLSEKEDAVNKIHTTGFKDQNEMLSSLQKLAVLKADLEKKKQSMGKLYSLKQDLLSTLKNKSVTQKTEAWLDNFARCWDNLVQKLEKSTAQISQAVTTTQPSLTQTTVMETVTTVTTREQILVKHAQEELPPPPPQKKRQITVDTLERLQELQEATDELDLKLRQAEVIKGSWQPVGDLLIDSLQDHLEKVKALRGEIAPLKENVSHVNDLARQLTTLGIQLSPYNLSTLEDLNTRWKLLQVAVEDRVRQLHEAHRDFGPASQHFLSTSVQGPWERAISPNKVPYYINHETQTTCWDHPKMTELYQSLADLNNVRFSAYRTAMKLRRLQKALCLDLLSLSAACDALDQHNLKQNDQPMDILQIINCLTTIYDRLEQEHNNLVNVPLCVDMCLNWLLNVYDTGRTGRIRVLSFKTGIISLCKAHLEDKYRYLFKQVASSTGFCDQRRLGLLLHDSIQIPRQLGEVASFGGSNIEPSVRSCFQFANNKPEIEAALFLDWMRLEPQSMVWLPVLHRVAAAETAKHQAKCNICKECPIIGFRYRSLKHFNYDICQSCFFSGRVAKGHKMHYPMVEYCTPTTSGEDVRDFAKVLKNKFRTKRYFAKHPRMGYLPVQTVLEGDNMETPVTLINFWPVDSAPASSPQLSHDDTHSRIEHYASRLAEMENSNGSYLNDSISPNESIDDEHLLIQHYCQSLNQDSPLSQPRSPAQILISLESEERGELERILADLEEENRNLQAEYDRLKQQHEHKGLSPLPSPPEMMPTSPQSPRDAELIAEAKLLRQHKGRLEARMQILEDHNKQLESQLHRLRQLLEQPQAEAKVNGTTVSSPSTSLQRSDSSQPMLLRVVGSQTSDSMGEEDLLSPPQDTSTGLEEVMEQLNNSFPSSRGRNTPGKPMREDTM

SEQ ID NO: 61 - DNA, 34 bp, synthetic construct
  source 1..34: mol_type = other DNA
cgctccatatttggcgggagttatttttagagcg

SEQ ID NO: 62 - DNA, 56 bp, synthetic construct
  source 1..56: mol_type = other DNA
ggacacccaaatatggcgacggttcctcacccgtcgctaaaaataactccgtgtcc

SEQ ID NO: 63 - DNA, 38 bp, synthetic construct
  source 1..38: mol_type = other DNA
gggagttatttttagagcggggagttatttttagagcg

SEQ ID NO: 64 - DNA, 52 bp, synthetic construct
  source 1..52: mol_type = other DNA
ggacacccaaatatggcgacggttcctcacggacacccaaatatggcgacgg

SEQ ID NO: 65 - DNA, 38 bp, synthetic construct
  source 1..38: mol_type = other DNA
cgctctaaaaataactcccgggagttatttttagagcg

SEQ ID NO: 66 - DNA, 52 bp, synthetic construct
  source 1..52: mol_type = other DNA
ggacacccaaatatggcgacggttcctcacccgtcggcatatttgggtgtcg

SEQ ID NO: 67 - DNA, 4017 bp, synthetic construct
  source 1..4017: mol_type = other DNA
atgctttggtgggaagaggtggaagattgctatgagagggaagatgtgcagaagaaaaccttcaccaaatgggtcaatgcccagttcagcaagtttggcaagcagcacattgagaacctgttcagtgacctgcaggatggcagaaggctgctggatctgctggaaggcctgacaggccagaagctgcctaaagagaagggcagcacaagagtgcatgccctgaacaatgtgaacaaggccctgagagtgctgcagaacaacaatgtggacctggtcaatattggcagcacagacattgtggatggcaaccacaagctgaccctgggcctgatctggaacatcatcctgcactggcaagtgaagaatgtgatgaagaacatcatggctggcctgcagcagaccaactctgagaagatcctgctgagctgggtcagacagagcaccagaaactaccctcaagtgaatgtgatcaacttcaccacctcttggagtgatggactggccctgaatgccctgatccacagccacagacctgacctgtttgactggaactctgttgtgtgccagcagtctgccacacagagactggaacatgccttcaacattgccagataccagctgggaattgagaaactgctggaccctgaggatgtggacaccacctatcctgacaagaaatccatcctcatgtacatcaccagcctgttccaggtgctgccccagcaagtgtccattgaggccattcaagaggttgagatgctgcccagacctcctaaagtgaccaaagaggaacacttccagctgcaccaccagatgcactactctcagcagatcacagtgtctctggcccagggatatgagagaacaagcagccccaagcctaggttcaagagctatgcctacacacaggctgcctatgtgaccacatctgaccccacaagaagcccatttccaagccagcatctggaagcccctgaggacaagagctttggcagcagcctgatggaatctgaagtgaacctggatagataccagacagccctggaagaagtgctgtcctggctgctgtctgctgaggatacactgcaggctcagggtgaaatcagcaatgatgtggaagtggtcaaggaccagtttcacacccatgagggctacatgatggacctgacagcccaccagggcagagtgggaaatatcctgcagctgggctccaagctgattggcacaggcaagctgtctgaggatgaagagacagaggtgcaagagcagatgaacctgctgaacagcagatgggagtgtctgagagtggccagcatggaaaagcagagcaacctgcacagagtgctcatggacctgcagaatcagaaactgaaagaactgaatgactggctgaccaagacagaagaaaggactaggaagatggaagaggaacctctgggaccagacctggaagatctgaaaagacaggtgcagcagcataaggtgctgcaagaggaccttgagcaagagcaagtcagagtgaacagcctgacacacatggtggtggttgtggatgagtcctctggggatcatgccacagctgctctggaagaacagctgaaggtgctgggagacagatgggccaacatctgtaggtggacagaggatagatgggtgctgctccaggacattctgctgaagtggcagagactgacagaggaacagtgcctgttttctgcctggctctctgagaaagaggatgctgtcaacaagatccataccacaggcttcaaggatcagaatgagatgctcagctccctgcagaaactggctgtgctgaaggctgacctggaaaagaaaaagcagtccatgggcaagctctacagcctgaagcaggacctgctgtctaccctgaagaacaagtctgtgacccagaaaactgaggcctggctggacaactttgctagatgctgggacaacctggtgcagaagctggaaaagtctacagcccagatcagccagcaacctgatcttgcccctggcctgaccacaattggagcctctccaacacagactgtgaccctggttacccagccagtggtcaccaaagagacagccatcagcaaactggaaatgcccagctctctgatgctggaagtccccacactggaaaggctgcaagaacttcaagaggccacagatgagctggacctgaagctgagacaggctgaagtgatcaaaggcagctggcagccagttggggacctgctcattgatagcctgcaggaccatctggaaaaagtgaaagccctgaggggagagattgcccctctgaaagaaaatgtgtcccatgtgaatgacctggccagacagctgaccacactgggaatccagctgagcccctacaacctgagcacccttgaggacctgaacaccaggtggaagctcctccaggtggcagtggaagatagagtcaggcagctgcatgaggcccacagagattttggaccagccagccagcactttctgtctacctctgtgcaaggcccctgggagagagctatctctcctaacaaggtgccctactacatcaaccatgagacacagaccacctgttgggatcaccccaagatgacagagctgtaccagagtctggcagacctcaacaatgtcagattcagtgcctacaggactgccatgaagctcagaaggctccagaaagctctgtgcctggacctgctttccctgagtgcagcttgtgatgccctggaccagcacaatctgaagcagaatgaccagcctatggacatcctccagatcatcaactgcctcaccaccatctatgataggctggaacaagagcacaacaatctggtcaatgtgcccctgtgtgtggacatgtgcctgaattggctgctgaatgtgtatgacacaggcagaacaggcaggatcagagtcctgtccttcaagacaggcatcatctccctgtgcaaagcccacttggaggacaagtacagatacctgttcaagcaagtggcctccagcacaggcttttgtgaccagagaaggctgggcctgctcctgcatgacagcattcagatccctagacagctgggagaagtggcttcctttggaggcagcaatattgagccatcagtcaggtcctgttttcagtttgccaacaacaagcctgagattgaggctgccctgttcctggactggatgagacttgagcctcagagcatggtctggctgcctgtgcttcatagagtggctgctgctgagactgccaagcaccaggccaagtgcaacatctgcaaagagtgccccatcattggcttcagatacagatccctgaagcacttcaactatgatatctgccagagctgcttctttagtggcagggttgccaagggccacaaaatgcactaccccatggtggaatactgcaccccaacaacctctggggaagatgttagagactttgccaaggtgctgaaaaacaagttcaggaccaagagatactttgctaagcaccccagaatgggctacctgcctgtccagacagtgcttgagggtgacaacatggaaacccctgtgacactgatcaatttctggccagtggactctgcccctgcctcaagtccacagctgtcccatgatgacacccacagcagaattgagcactatgcctccagactggcagagatggaaaacagcaatggcagctacctgaatgatagcatcagccccaatgagagcattgatgatgagcatctgctgatccagcactactgtcagtccctgaaccaggactctccactgagccagcctagaagccctgctcagatcctgatcagccttgagtctgaggaaaggggagagctggaaagaatcctggcagatcttgaggaagagaacagaaacctgcaggcagagtatgacaggctcaaacagcagcatgagcacaagggactgagccctctgccttctcctcctgaaatgatgcccacctctccacagtctccaaggtgatga

SEQ ID NO: 68 - DNA, 3573 bp, synthetic construct
  source 1..3573: mol_type = other DNA
atgctttggtgggaagaggtggaagattgctatgagagggaagatgtgcagaagaaaaccttcaccaaatgggtcaatgcccagttcagcaagtttggcaagcagcacattgagaacctgttcagtgacctgcaggatggcagaaggctgctggatctgctggaaggcctgacaggccagaagctgcctaaagagaagggcagcacaagagtgcatgccctgaacaatgtgaacaaggccctgagagtgctgcagaacaacaatgtggacctggtcaatattggcagcacagacattgtggatggcaaccacaagctgaccctgggcctgatctggaacatcatcctgcactggcaagtgaagaatgtgatgaagaacatcatggctggcctgcagcagaccaactctgagaagatcctgctgagctgggtcagacagagcaccagaaactaccctcaagtgaatgtgatcaacttcaccacctcttggagtgatggactggccctgaatgccctgatccacagccacagacctgacctgtttgactggaactctgttgtgtgccagcagtctgccacacagagactggaacatgccttcaacattgccagataccagctgggaattgagaaactgctggaccctgaggatgtggacaccacctatcctgacaagaaatccatcctcatgtacatcaccagcctgttccaggtgctgccccagcaagtgtccattgaggccattcaagaggttgagatgctgcccagacctcctaaagtgaccaaagaggaacacttccagctgcaccaccagatgcactactctcagcagatcacagtgtctctggcccagggatatgagagaacaagcagccccaagcctaggttcaagagctatgcctacacacaggctgcctatgtgaccacatctgaccccacaagaagcccatttccaagccagcatctggaagcccctgaggacaagagctttggcagcagcctgatggaatctgaagtgaacctggatagataccagacagccctggaagaagtgctgtcctggctgctgtctgctgaggatacactgcaggctcagggtgaaatcagcaatgatgtggaagtggtcaaggaccagtttcacacccatgagggctacatgatggacctgacagcccaccagggcagagtgggaaatatcctgcagctgggctccaagctgattggcacaggcaagctgtctgaggatgaagagacagaggtgcaagagcagatgaacctgctgaacagcagatgggagtgtctgagagtggccagcatggaaaagcagagcaacctgcacagagtgctcatggacctgcagaatcagaaactgaaagaactgaatgactggctgaccaagacagaagaaaggactaggaagatggaagaggaacctctgggaccagacctggaagatctgaaaagacaggtgcagcagcataaggtgctgcaagaggaccttgagcaagagcaagtcagagtgaacagcctgacacacatggtggtggttgtggatgagtcctctggggatcatgccacagctgctctggaagaacagctgaaggtgctgggagacagatgggccaacatctgtaggtggacagaggatagatgggtgctgctccaggacattctgctgaagtggcagagactgacagaggaacagtgcctgttttctgcctggctctctgagaaagaggatgctgtcaacaagatccataccacaggcttcaaggatcagaatgagatgctcagctccctgcagaaactggctgtgctgaaggctgacctggaaaagaaaaagcagtccatgggcaagctctacagcctgaagcaggacctgctgtctaccctgaagaacaagtctgtgacccagaaaactgaggcctggctggacaactttgctagatgctgggacaacctggtgcagaagctggaaaagtctacagcccagatcagccagcaacctgatcttgcccctggcctgaccacaattggagcctctccaacacagactgtgaccctggttacccagccagtggtcaccaaagagacagccatcagcaaactggaaatgcccagctctctgatgctggaagtccccacactggaaaggctgcaagaacttcaagaggccacagatgagctggacctgaagctgagacaggctgaagtgatcaaaggcagctggcagccagttggggacctgctcattgatagcctgcaggaccatctggaaaaagtgaaagccctgaggggagagattgcccctctgaaagaaaatgtgtcccatgtgaatgacctggccagacagctgaccacactgggaatccagctgagcccctacaacctgagcacccttgaggacctgaacaccaggtggaagctcctccaggtggcagtggaagatagagtcaggcagctgcatgaggcccacagagattttggaccagccagccagcactttctgtctacctctgtgcaaggcccctgggagagagctatctctcctaacaaggtgccctactacatcaaccatgagacacagaccacctgttgggatcaccccaagatgacagagctgtaccagagtctggcagacctcaacaatgtcagattcagtgcctacaggactgccatgaagctcagaaggctccagaaagctctgtgcctggacctgctttccctgagtgcagcttgtgatgccctggaccagcacaatctgaagcagaatgaccagcctatggacatcctccagatcatcaactgcctcaccaccatctatgataggctggaacaagagcacaacaatctggtcaatgtgcccctgtgtgtggacatgtgcctgaattggctgctgaatgtgtatgacacaggcagaacaggcaggatcagagtcctgtccttcaagacaggcatcatctccctgtgcaaagcccacttggaggacaagtacagatacctgttcaagcaagtggcctccagcacaggcttttgtgaccagagaaggctgggcctgctcctgcatgacagcattcagatccctagacagctgggagaagtggcttcctttggaggcagcaatattgagccatcagtcaggtcctgttttcagtttgccaacaacaagcctgagattgaggctgccctgttcctggactggatgagacttgagcctcagagcatggtctggctgcctgtgcttcatagagtggctgctgctgagactgccaagcaccaggccaagtgcaacatctgcaaagagtgccccatcattggcttcagatacagatccctgaagcacttcaactatgatatctgccagagctgcttctttagtggcagggttgccaagggccacaaaatgcactaccccatggtggaatactgcaccccaacaacctctggggaagatgttagagactttgccaaggtgctgaaaaacaagttcaggaccaagagatactttgctaagcaccccagaatgggctacctgcctgtccagacagtgcttgagggtgacaacatggaaacc

SEQ ID NO: 69 - DNA, 3855 bp, synthetic construct
  source 1..3855: mol_type = other DNA
atgctttggtgggaagaggtggaagattgctatgagagggaagatgtgcagaagaaaaccttcaccaaatgggtcaatgcccagttcagcaagtttggcaagcagcacattgagaacctgttcagtgacctgcaggatggcagaaggctgctggatctgctggaaggcctgacaggccagaagctgcctaaagagaagggcagcacaagagtgcatgccctgaacaatgtgaacaaggccctgagagtgctgcagaacaacaatgtggacctggtcaatattggcagcacagacattgtggatggcaaccacaagctgaccctgggcctgatctggaacatcatcctgcactggcaagtgaagaatgtgatgaagaacatcatggctggcctgcagcagaccaactctgagaagatcctgctgagctgggtcagacagagcaccagaaactaccctcaagtgaatgtgatcaacttcaccacctcttggagtgatggactggccctgaatgccctgatccacagccacagacctgacctgtttgactggaactctgttgtgtgccagcagtctgccacacagagactggaacatgccttcaacattgccagataccagctgggaattgagaaactgctggaccctgaggatgtggacaccacctatcctgacaagaaatccatcctcatgtacatcaccagcctgttccaggtgctgccccagcaagtgtccattgaggccattcaagaggttgagatgctgcccagacctcctaaagtgaccaaagaggaacacttccagctgcaccaccagatgcactactctcagcagatcacagtgtctctggcccagggatatgagagaacaagcagccccaagcctaggttcaagagctatgcctacacacaggctgcctatgtgaccacatctgaccccacaagaagcccatttccaagccagcatctggaagcccctgaggacaagagctttggcagcagcctgatggaatctgaagtgaacctggatagataccagacagccctggaagaagtgctgtcctggctgctgtctgctgaggatacactgcaggctcagggtgaaatcagcaatgatgtggaagtggtcaaggaccagtttcacacccatgagggctacatgatggacctgacagcccaccagggcagagtgggaaatatcctgcagctgggctccaagctgattggcacaggcaagctgtctgaggatgaagagacagaggtgcaagagcagatgaacctgctgaacagcagatgggagtgtctgagagtggccagcatggaaaagcagagcaacctgcacagagtgctcatggacctgcagaatcagaaactgaaagaactgaatgactggctgaccaagacagaagaaaggactaggaagatggaagaggaacctctgggaccagacctggaagatctgaaaagacaggtgcagcagcataaggtgctgcaagaggaccttgagcaagagcaagtcagagtgaacagcctgacacacatggtggtggttgtggatgagtcctctggggatcatgccacagctgctctggaagaacagctgaaggtgctgggagacagatgggccaacatctgtaggtggacagaggatagatgggtgctgctccaggacattctgctgaagtggcagagactgacagaggaacagtgcctgttttctgcctggctctctgagaaagaggatgctgtcaacaagatccataccacaggcttcaaggatcagaatgagatgctcagctccctgcagaaactggctgtgctgaaggctgacctggaaaagaaaaagcagtccatgggcaagctctacagcctgaagcaggacctgctgtctaccctgaagaacaagtctgtgacccagaaaactgaggcctggctggacaactttgctagatgctgggacaacctggtgcagaagctggaaaagtctacagcccagatcagccagcaacctgatcttgcccctggcctgaccacaattggagcctctccaacacagactgtgaccctggttacccagccagtggtcaccaaagagacagccatcagcaaactggaaatgcccagctctctgatgctggaagtccccacactggaaaggctgcaagaacttcaagaggccacagatgagctggacctgaagctgagacaggctgaagtgatcaaaggcagctggcagccagttggggacctgctcattgatagcctgcaggaccatctggaaaaagtgaaagccctgaggggagagattgcccctctgaaagaaaatgtgtcccatgtgaatgacctggccagacagctgaccacactgggaatccagctgagcccctacaacctgagcacccttgaggacctgaacaccaggtggaagctcctccaggtggcagtggaagatagagtcaggcagctgcatgaggcccacagagattttggaccagccagccagcactttctgtctacctctgtgcaaggcccctgggagagagctatctctcctaacaaggtgccctactacatcaaccatgagacacagaccacctgttgggatcaccccaagatgacagagctgtaccagagtctggcagacctcaacaatgtcagattcagtgcctacaggactgccatgaagctcagaaggctccagaaagctctgtgcctggacctgctttccctgagtgcagcttgtgatgccctggaccagcacaatctgaagcagaatgaccagcctatggacatcctccagatcatcaactgcctcaccaccatctatgataggctggaacaagagcacaacaatctggtcaatgtgcccctgtgtgtggacatgtgcctgaattggctgctgaatgtgtatgacacaggcagaacaggcaggatcagagtcctgtccttcaagacaggcatcatctccctgtgcaaagcccacttggaggacaagtacagatacctgttcaagcaagtggcctccagcacaggcttttgtgaccagagaaggctgggcctgctcctgcatgacagcattcagatccctagacagctgggagaagtggcttcctttggaggcagcaatattgagccatcagtcaggtcctgttttcagtttgccaacaacaagcctgagattgaggctgccctgttcctggactggatgagacttgagcctcagagcatggtctggctgcctgtgcttcatagagtggctgctgctgagactgccaagcaccaggccaagtgcaacatctgcaaagagtgccccatcattggcttcagatacagatccctgaagcacttcaactatgatatctgccagagctgcttctttagtggcagggttgccaagggccacaaaatgcactaccccatggtggaatactgcaccccaacaacctctggggaagatgttagagactttgccaaggtgctgaaaaacaagttcaggaccaagagatactttgctaagcaccccagaatgggctacctgcctgtccagacagtgcttgagggtgacaacatggaaacccctgtgacactgatcaatttctggccagtggactctgcccctgcctcaagtccacagctgtcccatgatgacacccacagcagaattgagcactatgcctccagactggcagagatggaaaacagcaatggcagctacctgaatgatagcatcagccccaatgagagcattgatgatgagcatctgctgatccagcactactgtcagtccctgaaccaggactctccactgagccagcctagaagccctgctcagatcctgatcagccttgagtcttgatga

SEQ ID NO: 70 - skipped

SEQ ID NO: 71 - DNA, 3581 bp, synthetic construct
  source 1..3581: mol_type = other DNA
atgctgtggtgggaggaggtggaggattgttatgaaagggaggacgtgcagaagaagacttttaccaagtgggtgaacgctcagttcagcaaatttgggaagcagcacatcgagaatctgttttccgacctgcaggatgggagacggctgctggatctgctggaaggactgactggccagaagctgcccaaagagaaggggagcactagggtgcacgccctgaacaacgtgaacaaagctctgagagtgctgcagaacaacaacgtggatctggtgaatattggcagtactgatatcgtggacgggaaccacaaactgacactgggcctgatctggaacattattctgcactggcaggtgaaaaatgtgatgaagaacatcatggccgggctgcagcagaccaattccgagaagatcctgctgtcttgggtgcggcagagcacccgcaactatccccaggtgaacgtgattaacttcactacatcctggagcgacgggctggccctgaatgctctgattcacagccacaggcctgatctgttcgactggaatagcgtggtgtgccagcagtctgccacacagcgcctggaacatgccttcaatatcgctcggtaccagctggggatcgaaaaactgctggacccagaggatgtggacactacatacccagataaaaagtctattctgatgtacattactagcctgttccaggtgctgccacagcaggtgtctattgaagccattcaggaggtggaaatgctgccccgcccccccaaagtgactaaagaggagcattttcagctgcatcatcagatgcattacagccagcagattaccgtgagcctggctcagggatatgagcgcaccagtagtccaaaaccacggttcaagtcctacgcttatacccaggctgcctacgtgacaactagcgaccctactagatccccctttccatcccagcacctggaggccccagaggacaagagctttgggtccagcctgatggaaagcgaggtgaatctggatcggtaccagacagccctggaggaggtgctgagctggctgctgagtgctgaagacacactgcaggcccagggcgaaatttccaatgacgtggaagtggtgaaggatcagttccacacacacgagggctatatgatggacctgacagctcaccaggggcgcgtgggcaatatcctgcagctgggctctaaactgatcggcaccgggaaactgagtgaggacgaggaaacagaagtgcaggagcagatgaacctgctgaacagccgctgggagtgtctgagagtggctagtatggagaagcagtccaacctgcaccgggtgctgatggacctgcagaaccagaaactgaaagagctgaacgactggctgacaaagactgaggaacgcacaaggaagatggaggaggagccactgggacccgacctggaggatctgaagagacaggtgcagcagcataaggtgctgcaggaggatctggaacaggagcaggtgcgggtgaactccctgacacatatggtggtggtggtggacgaatctagtggagatcacgccaccgccgccctggaggaacagctgaaggtgctgggggaccggtgggccaacatttgccggtggaccgaggacaggtgggtgctgctgcaggacatcctgctgaaatggcagaggctgaccgaggagcagtgtctgtttagtgcttggctgagcgagaaagaggacgccgtgaacaagatccacacaaccggctttaaggatcagaacgaaatgctgtctagcctgcagaaactggctgtgctgaaggccgatctggagaaaaagaagcagagcatgggcaaactgtatagcctgaaacaggacctgctgagcaccctgaagaacaagagcgtgacccagaagacagaagcctggctggataactttgcccgctgctgggacaacctggtgcagaaactggagaaaagtacagctcagatctctcaggctgtgaccacaacccagcctagcctgacccagacaaccgtgatggaaaccgtgaccaccgtgacaacccgcgaacagatcctggtgaaacatgcccaggaagagctgccacctccacctccccagaagaagagaaccctggagcggctgcaggagctgcaggaagccactgacgaactggacctgaagctgaggcaggccgaagtgattaaggggtcttggcagcctgtgggcgatctgctgattgattccctgcaggaccacctggaaaaggtgaaggctctgagaggcgaaattgctccactgaaggagaacgtgagtcatgtgaacgatctggctagacagctgacaacactgggcatccagctgagcccatacaatctgagcacactggaggacctgaataccaggtggaagctgctgcaggtggctgtggaagaccgggtgcggcagctgcatgaggcccatcgcgacttcggaccagccagccagcactttctgagcacatccgtgcaggggccctgggagagggccatttctcccaacaaggtgccctactatattaatcacgagacccagaccacttgttgggaccatcccaagatgacagaactgtaccagtccctggccgatctgaacaacgtgaggtttagcgcttacagaaccgctatgaagctgagacggctgcagaaggccctgtgcctggatctgctgtccctgtccgccgcctgcgatgccctggatcagcataatctgaagcagaacgatcagccaatggatatcctgcagatcatcaactgcctgaccactatctacgacaggctggagcaggagcacaacaacctggtgaacgtgcctctgtgcgtggatatgtgcctgaactggctgctgaacgtgtatgacactgggcgcaccggccggatcagagtgctgagttttaaaactgggattatctccctgtgtaaggcccacctggaggacaagtacaggtacctgttcaagcaggtggctagtagcactggattttgtgaccagcgccgcctgggactgctgctgcatgatagtatccagattcctagacagctgggagaggtggctagtttcggaggatctaacatcgaacccagcgtgcgcagctgtttccagtttgccaataacaaacctgaaatcgaggctgctctgttcctggattggatgcgcctggaaccacagagcatggtgtggctgcctgtgctgcacagagtggctgccgccgaaactgccaagcaccaggctaaatgcaacatctgcaaggaatgtcccattatcggctttcgctacaggagtctgaaacattttaactacgatatttgccagagctgcttcttttccggaagagtggccaaaggacacaagatgcactaccctatggtggaatattgcaccccaactacatctggcgaagatgtgcgcgattttgccaaggtgctgaagaataagtttcggactaagaggtacttcgccaagcacccccgcatggggtatctgccagtgcagacagtgctggaaggagacaatatggagaccgatacaatgtgagc

SEQ ID NO: 72 - protein, 1201 aa, synthetic construct
MLWWEEVEDCYEREDVQKKTFTKWVNAQFSKFGKQHIENLFSDLQDGRRLLDLLEGLTGQKLPKEKGSTRVHALNNVNKALRVLQNNNVDLVNIGSTDIVDGNHKLTLGLIWNIILHWQVKNVMKNIMAGLQQTNSEKILLSWVRQSTRNYPQVNVINFTTSWSDGLALNALIHSHRPDLFDWNSVVCQQSATQRLEHAFNIARYQLGIEKLLDPEDVDTTYPDKKSILMYITSLFQVLPQQVSIEAIQEVEMLPRPPKVTKEEHFQLHHQMHYSQQITVSLAQGYERTSSPKPRFKSYAYTQAAYVTTSDPTRSPFPSQHLEAPEDKSFGSSLMESEVNLDRYQTALEEVLSWLLSAEDTLQAQGEISNDVEVVKDQFHTHEGYMMDLTAHQGRVGNILQLGSKLIGTGKLSEDEETEVQEQMNLLNSRWECLRVASMEKQSNLHSYVPSTYLTEITHVSQALLEVEQLLNAPDLCAKDFEDLFKQEESLKNIKDSLQQSSGRIDIIHSKKTAALQSATPVERVKLQEALSQLDFQWEKVNKMYKDRQGRFDRSVEKWRRFHYDIKIFNQWLTEAEQFLRKTQIPENWEHAKYKWYLKELQDGIGQRQTWRTLNATGEEIIQQSSKTDASILQEKLGSLNLRWQEVCKQLSDRKKRLEEQSDQWKRLHLSLQELLVWLQLKDDELSRQAPIGGDFPAVQKQNDVHRAFKRELKTKEPVIMSTLETVRIFLTEQPLEGLEKLYQEPRELPPEERAQNVTRLLRKQAEEVNTEWEKLNLHSADWQRKIDETLERLQELQEATDELDLKLRQAEVIKGSWQPVGDLLIDSLQDHLEKVKALRGEIAPLKENVSHVNDLARQLTTLGIQLSPYNLSTLEDLNTRWKLLQVAVEDRVRQLHEAHRDFGPASQHFLSTSVQGPWERAISPNKVPYYINHETQTTCWDHPKMTELYQSLADLNNVRFSAYRTAMKLRRLQKALCLDLLSLSAACDALDQHNLKQNDQPMDILQIINCLTTIYDRLEQEHNNLVNVPLCVDMCLNWLLNVYDTGRTGRIRVLSFKTGIISLCKAHLEDKYRYLFKQVASSTGFCLHRVAAAETAKHQAKCNICKECPIIGFRYRSLKHFNYDICQSCFFSGRVAKGHKMHYPMVEYCTPTTSGEDVRDFAKVLKNKFRTKRYFAKHPRMGYLPVQTVLEGDNMETDTM